European Patent Application EP 4 339 294 A2, published March 20, 2024. Title: METHOD OF MODIFYING ISOELECTRIC POINT OF ANTIBODY VIA AMINO ACID SUBSTITUTION IN CDR. Applicant: CHUGAI SEIYAKU KABUSHIKI KAISHA. Application EP. The sequence listing filed with the application follows.

SEQUENCE LISTING (246 sequences)

SEQ ID NO: 1 - protein, 6 aa, Mus musculus
SDHAWS

SEQ ID NO: 2 - protein, 16 aa, Mus musculus
YISYSGITTYNPSLKS

SEQ ID NO: 3 - protein, 10 aa, Mus musculus
SLARTTAMDY

SEQ ID NO: 4 - protein, 11 aa, Mus musculus
RASQDISSYLN

SEQ ID NO: 5 - protein, 7 aa, Mus musculus
YTSRLHS

SEQ ID NO: 6 - protein, 9 aa, Mus musculus
QQGNTLPYT

SEQ ID NO: 7 - protein, 30 aa, Homo sapiens
QVQLQESGPGLVRPSQTLSLTCTVSGYSIT

SEQ ID NO: 8 - protein, 14 aa, Homo sapiens
WVRQPPGRGLEWIG

SEQ ID NO: 9 - protein, 32 aa, Homo sapiens
RVTMLRDTSKNQFSLRLSSVTAADTAVYYCAR

SEQ ID NO: 10 - protein, 11 aa, Homo sapiens
WGQGSLVTVSS

SEQ ID NO: 11 - protein, 23 aa, Homo sapiens
DIQMTQSPSSLSASVGDRVTITC

SEQ ID NO: 12 - protein, 15 aa, Homo sapiens
WYQQKPGKAPKLLIY

SEQ ID NO: 13 - protein, 32 aa, Homo sapiens
GVPSRFSGSGSGTDFTFTISSLQPEDIATYYC

SEQ ID NO: 14 - protein, 10 aa, Homo sapiens
FGQGTKVEIK

SEQ ID NO: 15 - protein, 448 aa, synthetic construct
  REGION 1..448: note = An artificially synthesized peptide sequence
QVQLQESGPGLVRPSQTLSLTCTVSGYSITSDHAWSWVRQPPGRGLEWIGYISYSGITTYNPSLKSRVTMLRDTSKNQFSLRLSSVTAADTAVYYCARSLARTTAMDYWGQGSLVTVSSASTKGPSVFPLAPSSKSTSGGTAALGCLVKDYFPEPVTVSWNSGALTSGVHTFPAVLQSSGLYSLSSVVTVPSSSLGTQTYICNVNHKPSNTKVDKKVEPKSCDKTHTCPPCPAPELLGGPSVFLFPPKPKDTLMISRTPEVTCVVVDVSHEDPEVKFNWYVDGVEVHNAKTKPREEQYNSTYRVVSVLTVLHQDWLNGKEYKCKVSNKALPAPIEKTISKAKGQPREPQVYTLPPSRDELTKNQVSLTCLVKGFYPSDIAVEWESNGQPENNYKTTPPVLDSDGSFFLYSKLTVDKSRWQQGNVFSCSVMHEALHNHYTQKSLSLSPG

SEQ ID NO: 16 - protein, 214 aa, synthetic construct [sequence omitted]

SEQ ID NO: 17 - protein, 119 aa, synthetic construct [sequence omitted]

SEQ ID NO: 18 - protein, 107 aa, synthetic construct [sequence omitted]

SEQ ID NO: 19 - protein, 330 aa, Homo sapiens [sequence omitted]

SEQ ID NO: 20 - protein, 326 aa, Homo sapiens
ASTKGPSVFPLAPCSRSTSESTAALGCLVKDYFPEPVTVSWNSGALTSGVHTFPAVLQSSGLYSLSSVVTVPSSNFGTQTYTCNVDHKPSNTKVDKTVERKCCVECPPCPAPPVAGPSVFLFPPKPKDTLMISRTPEVTCVVVDVSHEDPEVQFNWYVDGVEVHNAKTKPREEQFNSTFRVVSVLTVVHQDWLNGKEYKCKVSNKGLPAPIEKTISKTKGQPREPQVYTLPPSREEMTKNQVSLTCLVKGFYPSDIAVEWESNGQPENNYKTTPPMLDSDGSFFLYSKLTVDKSRWQQGNVFSCSVMHEALHNHYTQKSLSLSPGK

SEQ ID NO: 21 - protein, 327 aa, Homo sapiens
ASTKGPSVFPLAPCSRSTSESTAALGCLVKDYFPEPVTVSWNSGALTSGVHTFPAVLQSSGLYSLSSVVTVPSSSLGTKTYTCNVDHKPSNTKVDKRVESKYGPPCPPCPAPEFLGGPSVFLFPPKPKDTLMISRTPEVTCVVVDVSQEDPEVQFNWYVDGVEVHNAKTKPREEQFNSTYRVVSVLTVLHQDWLNGKEYKCKVSNKGLPSSIEKTISKAKGQPREPQVYTLPPSQEEMTKNQVSLTCLVKGFYPSDIAVEWESNGQPENNYKTTPPVLDSDGSFFLYSRLTVDKSRWQEGNVFSCSVMHEALHNHYTQKSLSLSLGK

SEQ ID NO: 22 - protein, 119 aa, synthetic construct
  REGION 1..119: note = An artificially synthesized peptide sequence
QVQLQESGPGLVKPSETLSLTCAVSGYSISDDHAWSWVRQPPGEGLEWIGYISYSGITNYNPSLKGRVTISRDTSKNQFSLKLSSVTAADTAAYYCARVLARITAMDYWGEGTLVTVSS

SEQ ID NO: 23 - protein, 107 aa, synthetic construct
  REGION 1..107: note = An artificially synthesized peptide sequence
DIQMTQSPSSLSASVGDSVTITCQASQDISSYLNWYQQKPGKAPELLIYYGSELHSGVPSRFSGSGSGTDFTFTISSLEAEDAATYYCGQGNRLPYTFGQGTKVEIE

SEQ ID NO: 24 - protein, 324 aa, synthetic construct
  REGION 1..324: note = An artificially synthesized peptide sequence
ASTKGPSVFPLAPSSKSTSGGTAALGCLVKDYFPEPVTVSWNSGALTSGVHTFPAVLQSSGLYSLSSVVTVPSSNFGTQTYTCNVDHKPSNTKVDKTVERKSCVECPPCPAPPVAGPSVFLFPPKPKDTLMISRTPEVTCVVVDVSHEDPEVQFNWYVDGVEVHNAKTKPREEQFNSTFRVVSVLTVVHQDWLNGKEYKCKVSNKGLPSSIEKTISKAKGQPREPQVYTLPPSREEMTKNQVSLTCLVKGFYPSDIAVEWESNGQPENNYKTTPPVLDSDGSFFLYSKLTVDKSRWQQGNVFSCSVMHEALHNHYTQKSLSLSP

SEQ ID NO: 25 - protein, 324 aa, synthetic construct
  REGION 1..324: note = An artificially synthesized peptide sequence
ASTKGPSVFPLAPSSKSTSGGTAALGCLVKDYFPEPVTVSWNSGALTSGVHTFPAVLQSSGLYSLSSVVTVPSSSLGTKTYTCNVDHKPSNTKVDKTVERKSCVECPPCPAPPVAGPSVFLFPPKPKDTLMISRTPEVTCVVVDVSQEDPEVQFNWYVDGVEVHNAKTKPREEQFNSTYRVVSVLTVLHQDWLNGKEYKCKVSNKGLPSSIEKTISKAKGQPREPQVYTLPPSQEEMTKNQVSLTCLVKGFYPSDIAVEWESNGQPENNYKTTPPVLDSDGSFFLYSKLTVDKSRWQEGNVFSCSVMHEALHNHYTQKSLSLSL

SEQ ID NO: 26 - protein, 6 aa, synthetic construct
  REGION 1..6: note = An artificially synthesized peptide sequence
WDHAWS

SEQ ID NO: 27 - protein, 6 aa, synthetic construct
  REGION 1..6: note = An artificially synthesized peptide sequence
TDHAWS

SEQ ID NO: 28 - protein, 6 aa, synthetic construct
  REGION 1..6: note = An artificially synthesized peptide sequence
DDHAWS

SEQ ID NO: 29 - protein, 6 aa, synthetic construct
  REGION 1..6: note = An artificially synthesized peptide sequence
NDHAWS

SEQ ID NO: 30 - protein, 6 aa, synthetic construct
  REGION 1..6: note = An artificially synthesized peptide sequence
RDHAWS

SEQ ID NO: 31 - protein, 6 aa, synthetic construct
  REGION 1..6: note = An artificially synthesized peptide sequence
VDHAWS

SEQ ID NO: 32 - protein, 6 aa, synthetic construct
  REGION 1..6: note = An artificially synthesized peptide sequence
FDHAWS

SEQ ID NO: 33 - protein, 6 aa, synthetic construct
  REGION 1..6: note = An artificially synthesized peptide sequence
ADHAWS

SEQ ID NO: 34 - protein, 6 aa, synthetic construct
  REGION 1..6: note = An artificially synthesized peptide sequence
QDHAWS

SEQ ID NO: 35 - protein, 6 aa, synthetic construct
  REGION 1..6: note = An artificially synthesized peptide sequence
YDHAWS

SEQ ID NO: 36 - protein, 6 aa, synthetic construct
  REGION 1..6: note = An artificially synthesized peptide sequence
LDHAWS

SEQ ID NO: 37 - protein, 6 aa, synthetic construct
  REGION 1..6: note = An artificially synthesized peptide sequence
HDHAWS

SEQ ID NO: 38 - protein, 6 aa, synthetic construct
  REGION 1..6: note = An artificially synthesized peptide sequence
EDHAWS

SEQ ID NO: 39 - protein, 6 aa, synthetic construct
  REGION 1..6: note = An artificially synthesized peptide sequence
CDHAWS

SEQ ID NO: 40 - protein, 6 aa, synthetic construct
  REGION 1..6: note = An artificially synthesized peptide sequence
SDHAIS

SEQ ID NO: 41 - protein, 6 aa, synthetic construct
  REGION 1..6: note = An artificially synthesized peptide sequence
SDHAVS

SEQ ID NO: 42 - protein, 16 aa, synthetic construct
  REGION 1..16: note = An artificially synthesized peptide sequence
FISYSGITTYNPSLKS

SEQ ID NO: 43 - protein, 16 aa, synthetic construct
  REGION 1..16: note = An artificially synthesized peptide sequence
YISYSGIRTYNPSLKS

SEQ ID NO: 44 - protein, 16 aa, synthetic construct
  REGION 1..16: note = An artificially synthesized peptide sequence
YISYSGITSYNPSLKS

SEQ ID NO: 45 - protein, 16 aa, synthetic construct
  REGION 1..16: note = An artificially synthesized peptide sequence
YISYSGITNYNPSLKS

SEQ ID NO: 46 - protein, 10 aa, synthetic construct
  REGION 1..10: note = An artificially synthesized peptide sequence
ILARTTAMDY

SEQ ID NO: 47 - protein, 10 aa, synthetic construct
  REGION 1..10: note = An artificially synthesized peptide sequence
VLARTTAMDY

SEQ ID NO: 48 - protein, 10 aa, synthetic construct
  REGION 1..10: note = An artificially synthesized peptide sequence
TLARTTAMDY

SEQ ID NO: 49 - protein, 10 aa, synthetic construct
  REGION 1..10: note = An artificially synthesized peptide sequence
LLARTTAMDY

SEQ ID NO: 50 - protein, 10 aa, synthetic construct
  REGION 1..10: note = An artificially synthesized peptide sequence
STARTTAMDY

SEQ ID NO: 51 - protein, 10 aa, synthetic construct
  REGION 1..10: note = An artificially synthesized peptide sequence
SLARATAMDY

SEQ ID NO: 52 - protein, 10 aa, synthetic construct
  REGION 1..10: note = An artificially synthesized peptide sequence
SLARITAMDY

SEQ ID NO: 53 - protein, 10 aa, synthetic construct
  REGION 1..10: note = An artificially synthesized peptide sequence
SLARSTAMDY

SEQ ID NO: 54 - protein, 10 aa, synthetic construct
  REGION 1..10: note = An artificially synthesized peptide sequence
SLARTTSMDY

SEQ ID NO: 55 - protein, 10 aa, synthetic construct
  REGION 1..10: note = An artificially synthesized peptide sequence
SLARTTVMDY

SEQ ID NO: 56 - protein, 10 aa, synthetic construct
  REGION 1..10: note = An artificially synthesized peptide sequence
SLARTTALDY

SEQ ID NO: 57 - protein, 10 aa, synthetic construct
  REGION 1..10: note = An artificially synthesized peptide sequence
LLARATAMDY

SEQ ID NO: 58 - protein, 10 aa, synthetic construct
  REGION 1..10: note = An artificially synthesized peptide sequence
VLARATAMDY

SEQ ID NO: 59 - protein, 10 aa, synthetic construct
  REGION 1..10: note = An artificially synthesized peptide sequence
ILARATAMDY

SEQ ID NO: 60 - protein, 10 aa, synthetic construct
  REGION 1..10: note = An artificially synthesized peptide sequence
TLARATAMDY

SEQ ID NO: 61 - protein, 10 aa, synthetic construct
  REGION 1..10: note = An artificially synthesized peptide sequence
VLARITAMDY

SEQ ID NO: 62 - protein, 10 aa, synthetic construct
  REGION 1..10: note = An artificially synthesized peptide sequence
ILARITAMDY

SEQ ID NO: 63 - protein, 10 aa, synthetic construct
  REGION 1..10: note = An artificially synthesized peptide sequence
TLARITAMDY

SEQ ID NO: 64 - protein, 10 aa, synthetic construct
  REGION 1..10: note = An artificially synthesized peptide sequence
LLARITAMDY

SEQ ID NO: 65 - protein, 10 aa, synthetic construct
  REGION 1..10: note = An artificially synthesized peptide sequence
STARTTVLDY

SEQ ID NO: 66 - protein, 11 aa, synthetic construct
  REGION 1..11: note = An artificially synthesized peptide sequence
FASQDISSYLN

SEQ ID NO: 67 - protein, 11 aa, synthetic construct
  REGION 1..11: note = An artificially synthesized peptide sequence
RASRDISSYLN

SEQ ID NO: 68 - protein, 11 aa, synthetic construct
  REGION 1..11: note = An artificially synthesized peptide sequence
RASTDISSYLN

SEQ ID NO: 69 - protein, 11 aa, synthetic construct
  REGION 1..11: note = An artificially synthesized peptide sequence
RASQDISSFLN

SEQ ID NO: 70 - protein, 11 aa, synthetic construct
  REGION 1..11: note = An artificially synthesized peptide sequence
RASQDISSYLS

SEQ ID NO: 71 - protein, 7 aa, synthetic construct
  REGION 1..7: note = An artificially synthesized peptide sequence
YGSRLHS

SEQ ID NO: 72 - protein, 9 aa, synthetic construct
  REGION 1..9: note = An artificially synthesized peptide sequence
GQGNTLPYT

SEQ ID NO: 73 - protein, 9 aa, synthetic construct
  REGION 1..9: note = An artificially synthesized peptide sequence
NQGNTLPYT

SEQ ID NO: 74 - protein, 9 aa, synthetic construct
  REGION 1..9: note = An artificially synthesized peptide sequence
SQGNTLPYT

SEQ ID NO: 75 - protein, 9 aa, synthetic construct
  REGION 1..9: note = An artificially synthesized peptide sequence
QQSNTLPYT

SEQ ID NO: 76 - protein, 9 aa, synthetic construct
  REGION 1..9: note = An artificially synthesized peptide sequence
QQGNRLPYT

SEQ ID NO: 77 - protein, 9 aa, synthetic construct
  REGION 1..9: note = An artificially synthesized peptide sequence
QQGNSLPYT

SEQ ID NO: 78 - protein, 9 aa, synthetic construct
  REGION 1..9: note = An artificially synthesized peptide sequence
GQGNSLPYT

SEQ ID NO: 79 - protein, 9 aa, synthetic construct
  REGION 1..9: note = An artificially synthesized peptide sequence
GQGNRLPYT

SEQ ID NO: 80 - protein, 30 aa, synthetic construct
  REGION 1..30: note = An artificially synthesized peptide sequence
QVQLQESGPGLVKPSQTLSLTCTVSGYSIT

SEQ ID NO: 81 - protein, 30 aa, synthetic construct
  REGION 1..30: note = An artificially synthesized peptide sequence
QVQLQESGPGLVRPSETLSLTCTVSGYSIT

SEQ ID NO: 82 - protein, 30 aa, synthetic construct
  REGION 1..30: note = An artificially synthesized peptide sequence
QVQLQESGPGLVRPSQTLSLTCAVSGYSIT

SEQ ID NO: 83 - protein, 30 aa, synthetic construct
  REGION 1..30: note = An artificially synthesized peptide sequence
QVQLQESGPGLVRPSQTLSLTCTVSGYSIS

SEQ ID NO: 84 - protein, 30 aa, synthetic construct
  REGION 1..30: note = An artificially synthesized peptide sequence
QVQLQESGPGLVKPSETLSLTCAVSGYSIS

SEQ ID NO: 85 - protein, 14 aa, synthetic construct
  REGION 1..14: note = An artificially synthesized peptide sequence
WVRQPPGEGLEWIG

SEQ ID NO: 86 - protein, 32 aa, synthetic construct
  REGION 1..32: note = An artificially synthesized peptide sequence
RVTILRDTSKNQFSLRLSSVTAADTAVYYCAR

SEQ ID NO: 87 - protein, 32 aa, synthetic construct
  REGION 1..32: note = An artificially synthesized peptide sequence
RVTMSRDTSKNQFSLRLSSVTAADTAVYYCAR

SEQ ID NO: 88 - protein, 32 aa, synthetic construct
  REGION 1..32: note = An artificially synthesized peptide sequence
RVTMLRDTSKNQFSLKLSSVTAADTAVYYCAR

SEQ ID NO: 89 - protein, 32 aa, synthetic construct
  REGION 1..32: note = An artificially synthesized peptide sequence
RVTMLRDTSKNQFSLRLSSVTAADTAAYYCAR

SEQ ID NO: 90 - protein, 32 aa, synthetic construct
  REGION 1..32: note = An artificially synthesized peptide sequence
RVTISRDTSKNQFSLKLSSVTAADTAAYYCAR

SEQ ID NO: 91 - protein, 11 aa, synthetic construct
  REGION 1..11: note = An artificially synthesized peptide sequence
WGEGSLVTVSS

SEQ ID NO: 92 - protein, 23 aa, synthetic construct
  REGION 1..23: note = An artificially synthesized peptide sequence
DIQMTQSPSSLSASVGDSVTITC

SEQ ID NO: 93 - protein, 15 aa, synthetic construct
  REGION 1..15: note = An artificially synthesized peptide sequence
WYQQKPGKAPELLIY

SEQ ID NO: 94 - protein, 32 aa, synthetic construct
  REGION 1..32: note = An artificially synthesized peptide sequence
GVPSRFSGSGSGTDFTFTISSLEPEDIATYYC

SEQ ID NO: 95 - protein, 32 aa, synthetic construct
  REGION 1..32: note = An artificially synthesized peptide sequence
GVPSRFSGSGSGTDFTFTISSLQAEDIATYYC

SEQ ID NO: 96 - protein, 32 aa, synthetic construct
  REGION 1..32: note = An artificially synthesized peptide sequence
GVPSRFSGSGSGTDFTFTISSLQPEDAATYYC

SEQ ID NO: 97 - protein, 32 aa, synthetic construct
  REGION 1..32: note = An artificially synthesized peptide sequence
GVPSRFSGSGSGTDFTFTISSLEAEDAATYYC

SEQ ID NO: 98 - protein, 10 aa, synthetic construct
  REGION 1..10: note = An artificially synthesized peptide sequence
FGQGTKVEIE

SEQ ID NO: 99 - protein, 16 aa, synthetic construct
  REGION 1..16: note = An artificially synthesized peptide sequence
YISYSGITTYNPSLKG

SEQ ID NO: 100 - protein, 16 aa, synthetic construct
  REGION 1..16: note = An artificially synthesized peptide sequence
YISYSGITNYNPSLKG

SEQ ID NO: 101 - protein, 11 aa, synthetic construct
  REGION 1..11: note = An artificially synthesized peptide sequence
QASQDISSYLN

SEQ ID NO: 102 - protein, 7 aa, synthetic construct
  REGION 1..7: note = An artificially synthesized peptide sequence
YTSELHS

SEQ ID NO: 103 - protein, 7 aa, synthetic construct
  REGION 1..7: note = An artificially synthesized peptide sequence
YGSELHS

SEQ ID NO: 104 - protein, 119 aa, synthetic construct
  REGION 1..119: note = An artificially synthesized peptide sequence
QVQLQESGPGLVKPSETLSLTCAVSGYSISDDHAWSWVRQPPGEGLEWIGYISYSGITNYNPSLKGRVTISRDTSKNQFSLKLSSVTAADTAAYYCARSLARTTAMDYWGEGTLVTVSS

SEQ ID NO: 105 - protein, 107 aa, synthetic construct
  REGION 1..107: note = An artificially synthesized peptide sequence
DIQMTQSPSSLSASVGDSVTITCQASQDISSYLNWYQQKPGKAPELLIYYGSELHSGVPSRFSGSGSGTDFTFTISSLEAEDAATYYCQQGNSLPYTFGQGTKVEIE

SEQ ID NO: 106 - protein, 15 aa, synthetic construct
  REGION 1..15: note = An artificially synthesized peptide sequence
GGGGSGGGGSGGGGS

SEQ ID NO: 107 - DNA, 414 bp, synthetic construct
  misc_feature 1..414: note = An artificially synthesized nucleotide sequence
  source 1..414: mol_type = other DNA
atgggatggagctgtatcatcctcttcttggtagcaacagctacaggtgtccactcccaggtccaactgcaggagagcggtccaggtcttgtgagacctagccagaccctgagcctgacctgcaccgtgtctggctactcaattaccagcgatcatgcctggagctgggttcgccagccacctggacgaggtcttgagtggattggatacattagttatagtggaatcacaacctataatccatctctcaaatccagagtgacaatgctgagagacaccagcaagaaccagttcagcctgagactcagcagcgtgacagccgccgacaccgcggtttattattgtgcaagatccctagctcggactacggctatggactactggggtcaaggcagcctcgtcacagtctcctca

SEQ ID NO: 108 - DNA, 378 bp, synthetic construct
  misc_feature 1..378: note = An artificially synthesized nucleotide sequence
  source 1..378: mol_type = other DNA
atgggatggagctgtatcatcctcttcttggtagcaacagctacaggtgtccactccgacatccagatgacccagagcccaagcagcctgagcgccagcgtgggtgacagagtgaccatcacctgtagagccagccaggacatcagcagttacctgaattggtaccagcagaagccaggaaaggctccaaagctgctgatctactacacctccagactgcactctggtgtgccaagcagattcagcggtagcggtagcggtaccgacttcaccttcaccatcagcagcctccagccagaggacatcgctacctactactgccaacagggtaacacgcttccatacacgttcggccaagggaccaaggtggaaatcaaa

SEQ ID NO: 109 - protein, 445 aa, synthetic construct
  REGION 1..445: note = An artificially synthesized peptide sequence
QVQLQESGPGLVRPSQTLSLTCTVSGYSITSDHAWSWVRQPPGRGLEWIGYISYSGITTYNPSLKSRVTMLRDTSKNQFSLRLSSVTAADTAVYYCARSLARTTAMDYWGQGSLVTVSSASTKGPSVFPLAPCSRSTSESTAALGCLVKDYFPEPVTVSWNSGALTSGVHTFPAVLQSSGLYSLSSVVTVPSSNFGTQTYTCNVDHKPSNTKVDKTVERKCCVECPPCPAPPVAGPSVFLFPPKPKDTLMISRTPEVTCVVVDVSHEDPEVQFNWYVDGVEVHNAKTKPREEQFNSTFRVVSVLTVVHQDWLNGKEYKCKVSNKGLPAPIEKTISKTKGQPREPQVYTLPPSREEMTKNQVSLTCLVKGFYPSDIAVEWESNGQPENNYKTTPPMLDSDGSFFLYSKLTVDKSRWQQGNVFSCSVMHEALHNHYTQKSLSLSPGK

SEQ ID NO: 110 - protein, 446 aa, synthetic construct
  REGION 1..446: note = An artificially synthesized peptide sequence
QVQLQESGPGLVRPSQTLSLTCTVSGYSITSDHAWSWVRQPPGRGLEWIGYISYSGITTYNPSLKSRVTMLRDTSKNQFSLRLSSVTAADTAVYYCARSLARTTAMDYWGQGSLVTVSSASTKGPSVFPLAPCSRSTSESTAALGCLVKDYFPEPVTVSWNSGALTSGVHTFPAVLQSSGLYSLSSVVTVPSSSLGTKTYTCNVDHKPSNTKVDKRVESKYGPPCPPCPAPEFLGGPSVFLFPPKPKDTLMISRTPEVTCVVVDVSQEDPEVQFNWYVDGVEVHNAKTKPREEQFNSTYRVVSVLTVLHQDWLNGKEYKCKVSNKGLPSSIEKTISKAKGQPREPQVYTLPPSQEEMTKNQVSLTCLVKGFYPSDIAVEWESNGQPENNYKTTPPVLDSDGSFFLYSRLTVDKSRWQEGNVFSCSVMHEALHNHYTQKSLSLSLGK

SEQ ID NO: 111 - protein, 445 aa, synthetic construct
  REGION 1..445: note = An artificially synthesized peptide sequence
QVQLQESGPGLVRPSQTLSLTCTVSGYSITSDHAWSWVRQPPGRGLEWIGYISYSGITTYNPSLKSRVTMLRDTSKNQFSLRLSSVTAADTAVYYCARSLARTTAMDYWGQGSLVTVSSASTKGPSVFPLAPCSRSTSESTAALGCLVKDYFPEPVTVSWNSGALTSGVHTFPAVLQSSGLYSLSSVVTVPSSNFGTQTYTCNVDHKPSNTKVDKTVERKCCVECPPCPAPPVAGPSVFLFPPKPKDTLMISRTPEVTCVVVDVSHEDPEVQFNWYVDGVEVHNAKTKPREEQFNSTFRVVSVLTVVHQDWLNGKEYKCKVSNKGLPAPIEKTISKTKGQPREPQVYTLPPSREEMTKNQVSLTCLVKGFYPSDIAVEWESNGQPENNYKTTPPVLDSDGSFFLYSKLTVDKSRWQQGNVFSCSVMHEALHNHYTQKSLSLSPGK

SEQ ID NO: 112 - protein, 446 aa, synthetic construct
  REGION 1..446: note = An artificially synthesized peptide sequence
QVQLQESGPGLVRPSQTLSLTCTVSGYSITSDHAWSWVRQPPGRGLEWIGYISYSGITTYNPSLKSRVTMLRDTSKNQFSLRLSSVTAADTAVYYCARSLARTTAMDYWGQGSLVTVSSASTKGPSVFPLAPCSRSTSESTAALGCLVKDYFPEPVTVSWNSGALTSGVHTFPAVLQSSGLYSLSSVVTVPSSSLGTKTYTCNVDHKPSNTKVDKRVESKYGPPCPPCPAPEFLGGPSVFLFPPKPKDTLMISRTPEVTCVVVDVSQEDPEVQFNWYVDGVEVHNAKTKPREEQFNSTYRVVSVLTVLHQDWLNGKEYKCKVSNKGLPSSIEKTISKAKGQPREPQVYTLPPSQEEMTKNQVSLTCLVKGFYPSDIAVEWESNGQPENNYKTTPPVLDSDGSFFLYSKLTVDKSRWQEGNVFSCSVMHEALHNHYTQKSLSLSLGK

SEQ ID NO: 113 - protein, 443 aa, synthetic construct
  REGION 1..443: note = An artificially synthesized peptide sequence
QVQLQESGPGLVRPSQTLSLTCTVSGYSITSDHAWSWVRQPPGRGLEWIGYISYSGITTYNPSLKSRVTMLRDTSKNQFSLRLSSVTAADTAVYYCARSLARTTAMDYWGQGSLVTVSSASTKGPSVFPLAPSSKSTSGGTAALGCLVKDYFPEPVTVSWNSGALTSGVHTFPAVLQSSGLYSLSSVVTVPSSNFGTQTYTCNVDHKPSNTKVDKTVERKSCVECPPCPAPPVAGPSVFLFPPKPKDTLMISRTPEVTCVVVDVSHEDPEVQFNWYVDGVEVHNAKTKPREEQFNSTFRVVSVLTVVHQDWLNGKEYKCKVSNKGLPSSIEKTISKAKGQPREPQVYTLPPSREEMTKNQVSLTCLVKGFYPSDIAVEWESNGQPENNYKTTPPVLDSDGSFFLYSKLTVDKSRWQQGNVFSCSVMHEALHNHYTQKSLSLSP

SEQ ID NO: 114 - protein, 443 aa, synthetic construct
  REGION 1..443: note = An artificially synthesized peptide sequence
QVQLQESGPGLVRPSQTLSLTCTVSGYSITSDHAWSWVRQPPGRGLEWIGYISYSGITTYNPSLKSRVTMLRDTSKNQFSLRLSSVTAADTAVYYCARSLARTTAMDYWGQGSLVTVSSASTKGPSVFPLAPSSKSTSGGTAALGCLVKDYFPEPVTVSWNSGALTSGVHTFPAVLQSSGLYSLSSVVTVPSSSLGTKTYTCNVDHKPSNTKVDKTVERKSCVECPPCPAPPVAGPSVFLFPPKPKDTLMISRTPEVTCVVVDVSQEDPEVQFNWYVDGVEVHNAKTKPREEQFNSTYRVVSVLTVLHQDWLNGKEYKCKVSNKGLPSSIEKTISKAKGQPREPQVYTLPPSQEEMTKNQVSLTCLVKGFYPSDIAVEWESNGQPENNYKTTPPVLDSDGSFFLYSKLTVDKSRWQEGNVFSCSVMHEALHNHYTQKSLSLSL

SEQ ID NO: 115 - protein, 446 aa, synthetic construct
  REGION 1..446: note = An artificially synthesized peptide sequence
QVQLQESGPGLVRPSQTLSLTCTVSGYSITSDHAWSWVRQPPGRGLEWIGYISYSGITTYNPSLKSRVTMLRDTSKNQFSLRLSSVTAADTAVYYCARSLARTTAMDYWGQGSLVTVSSASTKGPSVFPLAPSSKSTSGGTAALGCLVKDYFPEPVTVSWNSGALTSGVHTFPAVLQSSGLYSLSSVVTVPSSSLGTQTYICNVNHKPSNTKVDKKVEPKSCDKTHTCPPCPAPPVAGPSVFLFPPKPKDTLMISRTPEVTCVVVDVSHEDPEVKFNWYVDGVEVHNAKTKPREEQYNSTYRVVSVLTVLHQDWLNGKEYKCKVSNKGLPSSIEKTISKAKGQPREPQVYTLPPSRDELTKNQVSLTCLVKGFYPSDIAVEWESNGQPENNYKTTPPVLDSDGSFFLYSKLTVDKSRWQQGNVFSCSVMHEALHNHYTQKSLSLSP

SEQ ID NO: 116 - protein, 327 aa, synthetic construct
  REGION 1..327: note = An artificially synthesized peptide sequence
ASTKGPSVFPLAPSSKSTSGGTAALGCLVKDYFPEPVTVSWNSGALTSGVHTFPAVLQSSGLYSLSSVVTVPSSSLGTQTYICNVNHKPSNTKVDKKVEPKSCDKTHTCPPCPAPPVAGPSVFLFPPKPKDTLMISRTPEVTCVVVDVSHEDPEVKFNWYVDGVEVHNAKTKPREEQYNSTYRVVSVLTVLHQDWLNGKEYKCKVSNKGLPSSIEKTISKAKGQPREPQVYTLPPSRDELTKNQVSLTCLVKGFYPSDIAVEWESNGQPENNYKTTPPVLDSDGSFFLYSKLTVDKSRWQQGNVFSCSVMHEALHNHYTQKSLSLSP

SEQ ID NO: 117 - protein, 443 aa, synthetic construct
  REGION 1..443: note = An artificially synthesized peptide sequence
QVQLQESGPGLVKPSETLSLTCAVSGYSISDDHAWSWVRQPPGEGLEWIGYISYSGITNYNPSLKGRVTISRDTSKNQFSLKLSSVTAADTAAYYCARVLARITAMDYWGEGTLVTVSSASTKGPSVFPLAPSSKSTSGGTAALGCLVKDYFPEPVTVSWNSGALTSGVHTFPAVLQSSGLYSLSSVVTVPSSNFGTQTYTCNVDHKPSNTKVDKTVERKSCVECPPCPAPPVAGPSVFLFPPKPKDTLMISRTPEVTCVVVDVSHEDPEVQFNWYVDGVEVHNAKTKPREEQFNSTFRVVSVLTVVHQDWLNGKEYKCKVSNKGLPSSIEKTISKAKGQPREPQVYTLPPSREEMTKNQVSLTCLVKGFYPSDIAVEWESNGQPENNYKTTPPVLDSDGSFFLYSKLTVDKSRWQQGNVFSCSVMHEALHNHYTQKSLSLSP

SEQ ID NO: 118 - protein, 324 aa, synthetic construct
  REGION 1..324: note = An artificially synthesized peptide sequence
ASTKGPSVFPLAPSSKSTSGGTAALGCLVKDYFPEPVTVSWNSGALTSGVHTFPAVLQSSGLYSLSSVVTVPSSNFGTQTYTCNVDHKPSNTKVDKTVERKSCVECPPCPAPPVAGPSVFLFPPKPKDTLMISRTPEVTCVVVDVSHEDPEVQFNWYVDGVEVHNAKTKPREEQFNSTFRVVSVLTVVHQDWLNGKEYKCKVSNKGLPAPIEKTISKTKGQPREPQVYTLPPSREEMTKNQVSLTCLVKGFYPSDIAVEWESNGQPENNYKTTPPVLDSDGSFFLYSKLTVDKSRWQQGNVFSCSVMHEALHNHYTQKSLSLSP

SEQ ID NO: 119 - protein, 443 aa, synthetic construct
  REGION 1..443: note = An artificially synthesized peptide sequence
QVQLQESGPGLVRPSQTLSLTCTVSGYSITSDHAWSWVRQPPGRGLEWIGYISYSGITTYNPSLKSRVTMLRDTSKNQFSLRLSSVTAADTAVYYCARSLARTTAMDYWGQGSLVTVSSASTKGPSVFPLAPSSKSTSGGTAALGCLVKDYFPEPVTVSWNSGALTSGVHTFPAVLQSSGLYSLSSVVTVPSSNFGTQTYTCNVDHKPSNTKVDKTVERKSCVECPPCPAPPVAGPSVFLFPPKPKDTLMISRTPEVTCVVVDVSHEDPEVQFNWYVDGVEVHNAKTKPREEQFNSTFRVVSVLTVVHQDWLNGKEYKCKVSNKGLPAPIEKTISKTKGQPREPQVYTLPPSREEMTKNQVSLTCLVKGFYPSDIAVEWESNGQPENNYKTTPPVLDSDGSFFLYSKLTVDKSRWQQGNVFSCSVMHEALHNHYTQKSLSLSP

SEQ ID NO: 120 - protein, 445 aa, synthetic construct
  REGION 1..445: note = An artificially synthesized peptide sequence
QVQLQESGPGLVRPSQTLSLTCTVSGYSITSDHAWSWVRQPPGRGLEWIGYISYSGITTYNPSLKSRVTMLRDTSKNQFSLRLSSVTAADTAVYYCARSLARTTAMDYWGQGSLVTVSSASTKGPSVFPLAPSSKSTSESTAALGCLVKDYFPEPVTVSWNSGALTSGVHTFPAVLQSSGLYSLSSVVTVPSSNFGTQTYTCNVDHKPSNTKVDKTVERKSCVECPPCPAPPVAGPSVFLFPPKPKDTLMISRTPEVTCVVVDVSHEDPEVQFNWYVDGVEVHNAKTKPREEQFNSTFRVVSVLTVVHQDWLNGKEYKCKVSNKGLPAPIEKTISKTKGQPREPQVYTLPPSREEMTKNQVSLTCLVKGFYPSDIAVEWESNGQPENNYKTTPPMLDSDGSFFLYSKLTVDKSRWQQGNVFSCSVMHEALHNHYTQKSLSLSPGK

SEQ ID NO: 121 - protein, 16 aa, synthetic construct
  REGION 1..16: note = An artificially synthesized peptide sequence
YISYSGITTYNPSLQD

SEQ ID NO: 122 - protein, 16 aa, synthetic construct
  REGION 1..16: note = An artificially synthesized peptide sequence
YISYSGITNYNPSLQD

SEQ ID NO: 123 - protein, 11 aa, synthetic construct
  REGION 1..11: note = An artificially synthesized peptide sequence
RASEDISSYLN

SEQ ID NO: 124 - protein, 11 aa, synthetic construct
  REGION 1..11: note = An artificially synthesized peptide sequence
QASEDISSYLN

SEQ ID NO: 125 - protein, 7 aa, synthetic construct
  REGION 1..7: note = An artificially synthesized peptide sequence
YTSRLES

SEQ ID NO: 126 - protein, 7 aa, synthetic construct
  REGION 1..7: note = An artificially synthesized peptide sequence
YGSELES

SEQ ID NO: 127 - protein, 32 aa, synthetic construct
  REGION 1..32: note = An artificially synthesized peptide sequence
RVTISRDTSKNQFSLKLSSVTAADTAVYYCAR

SEQ ID NO: 128 - protein, 32 aa, Homo sapiens
RVTISRDNSKNTLYLQMNSLRAEDTAVYYCAR

SEQ ID NO: 129 - protein, 32 aa, Homo sapiens
RVTITRDTSTSTVYMELSSLRSEDTAVYYCAR

SEQ ID NO: 130 - protein, 11 aa, synthetic construct
  REGION 1..11: note = An artificially synthesized peptide sequence
WGQGILVTVSS

SEQ ID NO: 131 - protein, 11 aa, synthetic construct
  REGION 1..11: note = An artificially synthesized peptide sequence
WGEGILVTVSS

SEQ ID NO: 132 - protein, 11 aa, synthetic construct
  REGION 1..11: note = An artificially synthesized peptide sequence
WGQGTLVTVSS

SEQ ID NO: 133 - protein, 11 aa, synthetic construct
  REGION 1..11: note = An artificially synthesized peptide sequence
WGEGTLVTVSS

SEQ ID NO: 134 - protein, 449 aa, synthetic construct
  REGION 1..449: note = An artificially synthesized peptide sequence
QVQLQESGPGLVKPSETLSLTCAVSGYSISDDHAWSWVRQPPGEGLEWIGYISYSGITNYNPSLKGRVTISRDNSKNTLYLQMNSLRAEDTAVYYCARVLARITAMDYWGEGTLVTVSSASTKGPSVFPLAPSSKSTSGGTAALGCLVKDYFPEPVTVSWNSGALTSGVHTFPAVLQSSGLYSLSSVVTVPSSSLGTQTYICNVNHKPSNTKVDKKVEPKSCDKTHTCPPCPAPELLGGPSVFLFPPKPKDTLMISRTPEVTCVVVDVSHEDPEVKFNWYVDGVEVHNAKTKPREEQYNSTYRVVSVLTVLHQDWLNGKEYKCKVSNKALPAPIEKTISKAKGQPREPQVYTLPPSRDELTKNQVSLTCLVKGFYPSDIAVEWESNGQPENNYKTTPPVLDSDGSFFLYSKLTVDKSRWQQGNVFSCSVMHEALHNHYTQKSLSLSPGK

SEQ ID NO: 135 - protein, 449 aa, synthetic construct
  REGION 1..449: note = An artificially synthesized peptide sequence
QVQLQESGPGLVKPSETLSLTCAVSGYSISDDHAWSWVRQPPGEGLEWIGYISYSGITNYNPSLQDRVTISRDNSKNTLYLQMNSLRAEDTAVYYCARLLARATAMDYWGQGILVTVSSASTKGPSVFPLAPSSKSTSGGTAALGCLVKDYFPEPVTVSWNSGALTSGVHTFPAVLQSSGLYSLSSVVTVPSSSLGTQTYICNVNHKPSNTKVDKKVEPKSCDKTHTCPPCPAPELLGGPSVFLFPPKPKDTLMISRTPEVTCVVVDVSHEDPEVKFNWYVDGVEVHNAKTKPREEQYNSTYRVVSVLTVLHQDWLNGKEYKCKVSNKALPAPIEKTISKAKGQPREPQVYTLPPSRDELTKNQVSLTCLVKGFYPSDIAVEWESNGQPENNYKTTPPVLDSDGSFFLYSKLTVDKSRWQQGNVFSCSVMHEALHNHYTQKSLSLSPGK

SEQ ID NO: 136 - protein, 214 aa, synthetic construct
  REGION 1..214: note = An artificially synthesized peptide sequence
DIQMTQSPSSLSASVGDSVTITCQASEDISSYLNWYQQKPGKAPELLIYYGSELESGVPSRFSGSGSGTDFTFTISSLEAEDAATYYCGQGNRLPYTFGQGTKVEIERTVAAPSVFIFPPSDEQLKSGTASVVCLLNNFYPREAKVQWKVDNALQSGNSQESVTEQDSKDSTYSLSSTLTLSKADYEKHKVYACEVTHQGLSSPVTKSFNRGEC

SEQ ID NO: 137 - protein, 449 aa, synthetic construct
  REGION 1..449: note = An artificially synthesized peptide sequence
QVQLQESGPGLVKPSETLSLTCAVSGYSISDDHAVSWVRQPPGEGLEWIGFISYSGITNYNPTLQDRVTISRDNSKNTLYLQMNSLRAEDTAVYYCARLLARATAMDVWGEGTLVTVSSASTKGPSVFPLAPSSKSTSGGTAALGCLVKDYFPEPVTVSWNSGALTSGVHTFPAVLQSSGLYSLSSVVTVPSSSLGTQTYICNVNHKPSNTKVDKKVEPKSCDKTHTCPPCPAPELLGGPSVFLFPPKPKDTLMISRTPEVTCVVVDVSHEDPEVKFNWYVDGVEVHNAKTKPREEQYNSTYRVVSVLTVLHQDWLNGKEYKCKVSNKALPAPIEKTISKAKGQPREPQVYTLPPSRDELTKNQVSLTCLVKGFYPSDIAVEWESNGQPENNYKTTPPVLDSDGSFFLYSKLTVDKSRWQQGNVFSCSVMHEALHNHYTQKSLSLSPGK

SEQ ID NO: 138 - protein, 214 aa, synthetic construct
  REGION 1..214: note = An artificially synthesized peptide sequence
DIQMTQSPSSLSASVGDSVTITCQASQDISSYLNWYQQKPGKAPELLIYYGSELESGVPSRFSGSGSGTDFTFTISSLEAEDAATYYCGQGNRLPYTFGQGTKVEIERTVAAPSVFIFPPSDEQLKSGTASVVCLLNNFYPREAKVQWKVDNALQSGNSQESVTEQDSKDSTYSLSSTLTLSKADYEKHKVYACEVTHQGLSSPVTKSFNRGEC

SEQ ID NO: 139 - protein, 447 aa, synthetic construct
  REGION 1..447: note = An artificially synthesized peptide sequence
QVQLQESGPGLVKPSETLSLTCAVSGYSISDDHAVSWVRQPPGEGLEWIGFISYSGITNYNPTLQDRVTISRDNSKNTLYLQMNSLRAEDTAVYYCARLLARATAMDVWGEGTLVTVSSASTKGPSVFPLAPSSKSTSGGTAALGCLVKDYFPEPVTVSWNSGALTSGVHTFPAVLQSSGLYSLSSVVTVPSSSLGTQTYICNVNHKPSNTKVDKKVEPKSCDKTHTCPPCPAPELLGGPSVFLFPPKPKDTLMISRTPEVTCVVVDVSHEDPEVKFNWYVDGVEVHNAKTKPREEQYNSTYRVVSVLTVLHQDWLNGKEYKCKVSNKALPAPIEKTISKAKGQPREPQVYTLPPSRDELTKNQVSLTCLVKGFYPSDIAVEWESNGQPENNYKTTPPVLDSDGSFFLYSKLTVDKSRWQQGNVFSCSVMHEALHAHYTQKSLSLSP

SEQ ID NO: 140 - protein, 267 aa, Homo sapiens
AESHLSLLYHLTAVSSPAPGTPAFWVSGWLGPQQYLSYNSLRGEAEPCGAWVWENQVSWYWEKETTDLRIKEKLFLEAFKALGGKGPYTLQGLLGCELGPDNTSVPTAKFALNGEEFMNFDLKQGTWGGDWPEALAISQRWQQQDKAANKELTFLLFSCPHRLREHLERGRGNLEWKEPPSMRLKARPSSPGFSVLTCSAFSFYPPELQLRFLRNGLAAGTGQGDFGPNSDGSFHASSSLTVKSGDEHHYCCIVQHAGLAQPLRVEL

SEQ ID NO: 141 - protein, 99 aa, Homo sapiens [sequence omitted]

SEQ ID NO: 142 - protein, 443 aa, synthetic construct
  REGION 1..443: note = An artificially synthesized peptide sequence
QVQLQESGPGLVRPSQTLSLTCTVSGYSITSDHAWSWVRQPPGRGLEWIGYISYSGITTYNPSLKSRVTMLRDTSKNQFSLRLSSVTAADTAVYYCARSLARTTAMDYWGQGSLVTVSSASTKGPSVFPLAPSSKSTSGGTAALGCLVKDYFPEPVTVSWNSGALTSGVHTFPAVLQSSGLYSLSSVVTVPSSNFGTQTYTCNVDHKPSNTKVDKTVERKSCVECPPCPAPPVAGPSVFLFPPKPKDTLMISRTPEVTCVVVDVSQEDPEVQFNWYVDGVEVHNAKTKPREEQFNSTFRVVSVLTVVHQDWLNGKEYKCKVSNKGLPAPIEKTISKTKGQPREPQVYTLPPSQEEMTKNQVSLTCLVKGFYPSDIAVEWESNGQPENNYKTTPPMLDSDGSFFLYSKLTVDKSRWQEGNVFSCSVMHEALHNHYTQKSLSLSP

SEQ ID NO: 143 - protein, 449 aa, synthetic construct
  REGION 1..449: note = An artificially synthesized peptide sequence
QVQLQESGPGLVRPSQTLSLTCTVSGYSITSDHAWSWVRQPPGRGLEWIGYISYSGITTYNPSLKSRVTMLRDTSKNQFSLRLSSVTAADTAVYYCARSLARTTAMDYWGQGSLVTVSSASTKGPSVFPLAPSSKSTSGGTAALGCLVKDYFPEPVTVSWNSGALTSGVHTFPAVLQSSGLYSLSSVVTVPSSSLGTQTYICNVNHKPSNTKVDKKVEPKSCDKTHTCPPCPAPELLGGPSVFLFPPKPKDTLMISRTPEVTCVVVDVSHEDPEVKFNWYVDGVEVHNAKTKPREEQYNSTYRVVSVLTVLHQDWLNGKEYKCKVSNKALPAPIEKTISKAKGQPREPQVYTLPPSRDELTKNQVSLTCLVKGFYPSDIAVEWESNGQPENNYKTTPPVLDSDGSFFLYSKLTVDKSRWQQGNVFSCSVMHEALHAHYTQKSLSLSPGK

SEQ ID NO: 144 - protein, 443 aa, synthetic construct
  REGION 1..443: note = An artificially synthesized peptide sequence
QVQLQESGPGLVRPSQTLSLTCTVSGYSITSDHAWSWVRQPPGRGLEWIGYISYSGITTYNPSLKSRVTMLRDTSKNQFSLRLSSVTAADTAVYYCARSLARTTAMDYWGQGSLVTVSSASTKGPSVFPLAPSSKSTSGGTAALGCLVKDYFPEPVTVSWNSGALTSGVHTFPAVLQSSGLYSLSSVVTVPSSNFGTQTYTCNVDHKPSNTKVDKTVERKSCVECPPCPAPPVAGPSVFLFPPKPKDTLMISRTPEVTCVVVDVSQEDPEVQFNWYVDGVEVHNAKTKPREEQFNSTFRVVSVLTVVHQDWLNGKEYKCKVSNKGLPAPIEKTISKTKGQPREPQVYTLPPSQEEMTKNQVSLTCLVKGFYPSDIAVEWESNGQPENNYKTTPPMLDSDGSFFLYSKLTVDKSRWQEGNVFSCSVMHEALHAHYTQKSLSLSP

SEQ ID NO: 145 - protein, 119 aa, Mus musculus
QVQLQESGPGLVKPSETLSLTCAVSGYSISDDHAWSWVRQPPGEGLEWIGYISYSGITNYNPSLQDRVTISRDNSKNTLYLQMNSLRAEDTAVYYCARLLARATAMDYWGQGILVTVSS

SEQ ID NO: 146 - protein, 107 aa, Mus musculus
DIQMTQSPSSLSASVGDSVTITCQASEDISSYLNWYQQKPGKAPELLIYYGSELESGVPSRFSGSGSGTDFTFTISSLEAEDAATYYCGQGNRLPYTFGQGTKVEIE

SEQ ID NO: 147 - protein, 120 aa, Mus musculus
QVQLVQSGAEVKKPGASVKVSCKASGYTFTGYIMNWVRQAPGQGLEWMGLINPYNGGTSYNQKFKGRVTITADESTSTAYMELSSLRSEDTAVYYCARDGYDDGPYTMDYWGQGTLVTVS

SEQ ID NO: 148 - protein, 107 aa, Mus musculus
DIQMTQSPSSLSASVGDRVTITCRTSENIYSFLAWYQQKPGKAPKLLIYNAKTLAKGVPSRFSGSGSGTDFTLTISSLQPEDFATYYCQHHYESPLTFGGGTKVEIK

SEQ ID NO: 149 - protein, 122 aa, Mus musculus
EVQLLESGGGLVQPGGSLRLSCAASGFTFSSYAMSWVRQAPGKGLEWVSGITGSGGSTYYADSVKGRFTISRDNSKNTLYLQMNSLRAEDTAVYYCAKDPGTTVIMSWFDPWGQGTLVTVSS

SEQ ID NO: 150 - protein, 108 aa, Mus musculus
EIVLTQSPGTLSLSPGERATLSCRASQSVRGRYLAWYQQKPGQAPRLLIYGASSRATGIPDRFSGSGSGTDFTLTISRLEPEDFAVFYCQQYGSSPRTFGQGTKVEIK

SEQ ID NO: 151 - protein, 324 aa, synthetic construct
  REGION 1..324: note = An artificially synthesized peptide sequence
ASTKGPSVFPLAPSSKSTSGGTAALGCLVKDYFPEPVTVSWNSGALTSGVHTFPAVLQSSGLYSLSSVVTVPSSNFGTQTYTCNVDHKPSNTKVDKTVERKSCVECPPCPAPPVAGPSVFLFPPKPKDTLMISRTPEVTCVVVDVSQEDPEVQFNWYVDGVEVHNAKTKPREEQFNSTFRVVSVLTVVHQDWLNGKEYKCKVSNKGLPAPIEKTISKTKGQPREPQVYTLPPSQEEMTKNQVSLTCLVKGFYPSDIAVEWESNGQPENNYKTTPPMLDSDGSFFLYSKLTVDKSRWQEGNVFSCSVMHEALHNHYTQKSLSLSP

SEQ ID NO: 152 - protein, 330 aa, synthetic construct
  REGION 1..330: note = An artificially synthesized peptide sequence
ASTKGPSVFPLAPSSKSTSGGTAALGCLVKDYFPEPVTVSWNSGALTSGVHTFPAVLQSSGLYSLSSVVTVPSSSLGTQTYICNVNHKPSNTKVDKKVEPKSCDKTHTCPPCPAPELLGGPSVFLFPPKPKDTLMISRTPEVTCVVVDVSHEDPEVKFNWYVDGVEVHNAKTKPREEQYNSTYRVVSVLTVLHQDWLNGKEYKCKVSNKALPAPIEKTISKAKGQPREPQVYTLPPSRDELTKNQVSLTCLVKGFYPSDIAVEWESNGQPENNYKTTPPVLDSDGSFFLYSKLTVDKSRWQQGNVFSCSVMHEALHAHYTQKSLSLSPGK

SEQ ID NO: 153 - protein, 324 aa, synthetic construct
  REGION 1..324: note = An artificially synthesized peptide sequence
ASTKGPSVFPLAPSSKSTSGGTAALGCLVKDYFPEPVTVSWNSGALTSGVHTFPAVLQSSGLYSLSSVVTVPSSNFGTQTYTCNVDHKPSNTKVDKTVERKSCVECPPCPAPPVAGPSVFLFPPKPKDTLMISRTPEVTCVVVDVSQEDPEVQFNWYVDGVEVHNAKTKPREEQFNSTFRVVSVLTVVHQDWLNGKEYKCKVSNKGLPAPIEKTISKTKGQPREPQVYTLPPSQEEMTKNQVSLTCLVKGFYPSDIAVEWESNGQPENNYKTTPPMLDSDGSFFLYSKLTVDKSRWQEGNVFSCSVMHEALHAHYTQKSLSLSP

SEQ ID NO: 154 - protein, 326 aa, synthetic construct
  REGION 1..326: note = An artificially synthesized peptide sequence
ASTKGPSVFPLAPSSKSTSESTAALGCLVKDYFPEPVTVSWNSGALTSGVHTFPAVLQSSGLYSLSSVVTVPSSNFGTQTYTCNVDHKPSNTKVDKTVERKSCVECPPCPAPPVAGPSVFLFPPKPKDTLMISRTPEVTCVVVDVSHEDPEVQFNWYVDGVEVHNAKTKPREEQFNSTFRVVSVLTVVHQDWLNGKEYKCKVSNKGLPAPIEKTISKTKGQPREPQVYTLPPSREEMTKNQVSLTCLVKGFYPSDIAVEWESNGQPENNYKTTPPMLDSDGSFFLYSKLTVDKSRWQQGNVFSCSVMHEALHNHYTQKSLSLSPGK

SEQ ID NO: 155 - protein, 326 aa, synthetic construct
  REGION 1..326: note = An artificially synthesized peptide sequence
ASTKGPSVFPLAPCSRSTSESTAALGCLVKDYFPEPVTVSWNSGALTSGVHTFPAVLQSSGLYSLSSVVTVPSSNFGTQTYTCNVDHKPSNTKVDKTVERKSCVECPPCPAPPVAGPSVFLFPPKPKDTLMISRTPEVTCVVVDVSHEDPEVQFNWYVDGVEVHNAKTKPREEQFNSTFRVVSVLTVVHQDWLNGKEYKCKVSNKGLPAPIEKTISKTKGQPREPQVYTLPPSREEMTKNQVSLTCLVKGFYPSDIAVEWESNGQPENNYKTTPPMLDSDGSFFLYSKLTVDKSRWQQGNVFSCSVMHEALHNHYTQKSLSLSPGK

SEQ ID NO: 156 - protein, 326 aa, synthetic construct
  REGION 1..326: note = An artificially synthesized peptide sequence
ASTKGPSVFPLAPCSRSTSESTAALGCLVKDYFPEPVTVSWNSGALTSGVHTFPAVLQSSGLYSLSSVVTVPSSNFGTQTYTCNVDHKPSNTKVDKTVERKCSVECPPCPAPPVAGPSVFLFPPKPKDTLMISRTPEVTCVVVDVSHEDPEVQFNWYVDGVEVHNAKTKPREEQFNSTFRVVSVLTVVHQDWLNGKEYKCKVSNKGLPAPIEKTISKTKGQPREPQVYTLPPSREEMTKNQVSLTCLVKGFYPSDIAVEWESNGQPENNYKTTPPMLDSDGSFFLYSKLTVDKSRWQQGNVFSCSVMHEALHNHYTQKSLSLSPGK

SEQ ID NO: 157 - protein, 445 aa, synthetic construct
  REGION 1..445: note = An artificially synthesized peptide sequence
QVQLQESGPGLVRPSQTLSLTCTVSGYSITSDHAWSWVRQPPGRGLEWIGYISYSGITTYNPSLKSRVTMLRDTSKNQFSLRLSSVTAADTAVYYCARSLARTTAMDYWGQGSLVTVSSASTKGPSVFPLAPCSRSTSESTAALGCLVKDYFPEPVTVSWNSGALTSGVHTFPAVLQSSGLYSLSSVVTVPSSNFGTQTYTCNVDHKPSNTKVDKTVERKSCVECPPCPAPPVAGPSVFLFPPKPKDTLMISRTPEVTCVVVDVSHEDPEVQFNWYVDGVEVHNAKTKPREEQFNSTFRVVSVLTVVHQDWLNGKEYKCKVSNKGLPAPIEKTISKTKGQPREPQVYTLPPSREEMTKNQVSLTCLVKGFYPSDIAVEWESNGQPENNYKTTPPMLDSDGSFFLYSKLTVDKSRWQQGNVFSCSVMHEALHNHYTQKSLSLSPGK

SEQ ID NO: 158 - protein, 445 aa, synthetic construct
  REGION 1..445: note = An artificially synthesized peptide sequence
QVQLQESGPGLVRPSQTLSLTCTVSGYSITSDHAWSWVRQPPGRGLEWIGYISYSGITTYNPSLKSRVTMLRDTSKNQFSLRLSSVTAADTAVYYCARSLARTTAMDYWGQGSLVTVSSASTKGPSVFPLAPCSRSTSESTAALGCLVKDYFPEPVTVSWNSGALTSGVHTFPAVLQSSGLYSLSSVVTVPSSNFGTQTYTCNVDHKPSNTKVDKTVERKCSVECPPCPAPPVAGPSVFLFPPKPKDTLMISRTPEVTCVVVDVSHEDPEVQFNWYVDGVEVHNAKTKPREEQFNSTFRVVSVLTVVHQDWLNGKEYKCKVSNKGLPAPIEKTISKTKGQPREPQVYTLPPSREEMTKNQVSLTCLVKGFYPSDIAVEWESNGQPENNYKTTPPMLDSDGSFFLYSKLTVDKSRWQQGNVFSCSVMHEALHNHYTQKSLSLSPGK

SEQ ID NO: 159 - protein, 119 aa, synthetic construct
  REGION 1..119: note = An artificially synthesized peptide sequence
QVQLQESGPGLVKPSETLSLTCAVSGYSISDDHAWSWVRQPPGEGLEWIGYISYSGITNYNPSLKGRVTISRDNSKNTLYLQMNSLRAEDTAVYYCARVLARITAMDYWGEGTLVTVSS

SEQ ID NO: 160 - protein, 119 aa, synthetic construct; identical to SEQ ID NO: 145
  REGION 1..119: note = An artificially synthesized peptide sequence

SEQ ID NO: 161 - protein, 119 aa, synthetic construct
  REGION 1..119: note = An artificially synthesized peptide sequence
QVQLQESGPGLVKPSETLSLTCAVSGYSISDDHAVSWVRQPPGEGLEWIGFISYSGITNYNPTLQDRVTISRDNSKNTLYLQMNSLRAEDTAVYYCARLLARATAMDVWGEGTLVTVSS

SEQ ID NO: 162 - protein, 107 aa, synthetic construct; identical to SEQ ID NO: 146
  REGION 1..107: note = An artificially synthesized peptide sequence

SEQ ID NO: 163 - protein, 107 aa, synthetic construct
  REGION 1..107: note = An artificially synthesized peptide sequence
DIQMTQSPSSLSASVGDSVTITCQASQDISSYLNWYQQKPGKAPELLIYYGSELESGVPSRFSGSGSGTDFTFTISSLEAEDAATYYCGQGNRLPYTFGQGTKVEIE

SEQ ID NO: 164 - protein, 328 aa, synthetic construct
  REGION 1..328: note = An artificially synthesized peptide sequence
ASTKGPSVFPLAPSSKSTSGGTAALGCLVKDYFPEPVTVSWNSGALTSGVHTFPAVLQSSGLYSLSSVVTVPSSSLGTQTYICNVNHKPSNTKVDKKVEPKSCDKTHTCPPCPAPELLGGPSVFLFPPKPKDTLMISRTPEVTCVVVDVSHEDPEVKFNWYVDGVEVHNAKTKPREEQYNSTYRVVSVLTVLHQDWLNGKEYKCKVSNKALPAPIEKTISKAKGQPREPQVYTLPPSRDELTKNQVSLTCLVKGFYPSDIAVEWESNGQPENNYKTTPPVLDSDGSFFLYSKLTVDKSRWQQGNVFSCSVMHEALHAHYTQKSLSLSP

SEQ ID NO: 165 - protein, 6 aa, synthetic construct
  REGION 1..6: note = An artificially synthesized peptide sequence
DDHAVS

SEQ ID NO: 166 - protein, 16 aa, synthetic construct
  REGION 1..16: note = An artificially synthesized peptide sequence
FISYSGITNYNPTLQD

SEQ ID NO: 167 - protein, 10 aa, synthetic construct
  REGION 1..10: note = An artificially synthesized peptide sequence
LLARATAMDV

SEQ ID NO: 168 - protein, 7 aa, synthetic construct
  REGION 1..7: note = An artificially synthesized peptide sequence
YGSELES

SEQ ID NO: 169 - protein, 6 aa, synthetic construct
  REGION 1..6: note = An artificially synthesized peptide sequence
HDHAWS

SEQ ID NO: 170 - protein, 16 aa, synthetic construct
  REGION 1..16: note = An artificially synthesized peptide sequence
FISYSGITNYNPSLQG

SEQ ID NO: 171 - protein, 10 aa, synthetic construct
  REGION 1..10: note = An artificially synthesized peptide sequence
SLARTTAMDY

SEQ ID NO: 172 - protein, 11 aa, synthetic construct
  REGION 1..11: note = An artificially synthesized peptide sequence
QASTDISSHLN

SEQ ID NO: 173 - protein, 7 aa, synthetic construct
  REGION 1..7: note = An artificially synthesized peptide sequence
YGSHLLS

SEQ ID NO: 174 - protein, 16 aa, synthetic construct
  REGION 1..16: note = An artificially synthesized peptide sequence
FISYSGITNYNPTLQG

SEQ ID NO: 175 - protein, 11 aa, synthetic construct
  REGION 1..11: note = An artificially synthesized peptide sequence
QASRDISSHLN

SEQ ID NO: 176 - protein, 119 aa, synthetic construct
  REGION 1..119: note = An artificially synthesized peptide sequence
QVQLQESGPGLVKPSETLSLTCAVSGHSISHDHAWSWVRQPPGEGLEWIGFISYSGITNYNPSLQGRVTISRDNSKNTLYLQMNSLRAEDTAVYYCARSLARTTAMDYWGEGTLVTVSS

SEQ ID NO: 177 - protein, 107 aa, synthetic construct
  REGION 1..107: note = An artificially synthesized peptide sequence
DIQMTQSPSSLSASVGDSVTITCQASTDISSHLNWYQQKPGKAPELLIYYGSHLLSGVPSRFSGSGSGTDFTFTISSLEAEDAATYYCGQGNRLPYTFGQGTKVEIE

SEQ ID NO: 178 - protein, 119 aa, synthetic construct
  REGION 1..119: note = An artificially synthesized peptide sequence
QVQLQESGPGLVKPSETLSLTCAVSGHSISHDHAWSWVRQPPGEGLEWIGFISYSGITNYNPTLQGRVTISRDNSKNTLYLQMNSLRAEDTAVYYCARSLARTTAMDYWGEGTLVTVSS

SEQ ID NO: 179 - protein, 107 aa, synthetic construct
  REGION 1..107: note = An artificially synthesized peptide sequence
DIQMTQSPSSLSASVGDSVTITCQASRDISSHLNWYQQKPGKAPELLIYYGSHLLSGVPSRFSGSGSGTDFTFTISSLEAEDAATYYCGQGNRLPYTFGQGTKVEIE

SEQ ID NO: 180 - protein, 443 aa, synthetic construct
  REGION 1..443: note = An artificially synthesized peptide sequence
QVQLQESGPGLVKPSETLSLTCAVSGHSISHDHAWSWVRQPPGEGLEWIGFISYSGITNYNPSLQGRVTISRDNSKNTLYLQMNSLRAEDTAVYYCARSLARTTAMDYWGEGTLVTVSSASTKGPSVFPLAPSSKSTSGGTAALGCLVKDYFPEPVTVSWNSGALTSGVHTFPAVLQSSGLYSLSSVVTVPSSNFGTQTYTCNVDHKPSNTKVDKTVERKSCVECPPCPAPPVAGPSVFLFPPKPKDTLMISRTPEVTCVVVDVSQEDPEVQFNWYVDGVEVHNAKTKPREEQFNSTFRVVSVLTVVHQDWLNGKEYKCKVSNKGLPAPIEKTISKTKGQPREPQVYTLPPSQEEMTKNQVSLTCLVKGFYPSDIAVEWESNGQPENNYKTTPPMLDSDGSFFLYSKLTVDKSRWQEGNVFSCSVMHEALHAHYTQKSLSLSP

SEQ ID NO: 181 - protein, 214 aa, synthetic construct
  REGION 1..214: note = An artificially synthesized peptide sequence
DIQMTQSPSSLSASVGDSVTITCQASTDISSHLNWYQQKPGKAPELLIYYGSHLLSGVPSRFSGSGSGTDFTFTISSLEAEDAATYYCGQGNRLPYTFGQGTKVEIERTVAAPSVFIFPPSDEQLKSGTASVVCLLNNFYPREAKVQWKVDNALQSGNSQESVTEQDSKDSTYSLSSTLTLSKADYEKHKVYACEVTHQGLSSPVTKSFNRGEC

SEQ ID NO: 182 - protein, 443 aa, synthetic construct
  REGION 1..443: note = An artificially synthesized peptide sequence
QVQLQESGPGLVKPSETLSLTCAVSGHSISHDHAWSWVRQPPGEGLEWIGFISYSGITNYNPTLQGRVTISRDNSKNTLYLQMNSLRAEDTAVYYCARSLARTTAMDYWGEGTLVTVSSASTKGPSVFPLAPSSKSTSGGTAALGCLVKDYFPEPVTVSWNSGALTSGVHTFPAVLQSSGLYSLSSVVTVPSSNFGTQTYTCNVDHKPSNTKVDKTVERKSCVECPPCPAPPVAGPSVFLFPPKPKDTLMISRTPEVTCVVVDVSQEDPEVQFNWYVDGVEVHNAKTKPREEQFNSTFRVVSVLTVVHQDWLNGKEYKCKVSNKGLPAPIEKTISKTKGQPREPQVYTLPPSQEEMTKNQVSLTCLVKGFYPSDIAVEWESNGQPENNYKTTPPMLDSDGSFFLYSKLTVDKSRWQEGNVFSCSVMHEALHAHYTQKSLSLSP

SEQ ID NO: 183 - protein, 214 aa, synthetic construct
  REGION 1..214: note = An artificially synthesized peptide sequence
DIQMTQSPSSLSASVGDSVTITCQASRDISSHLNWYQQKPGKAPELLIYYGSHLLSGVPSRFSGSGSGTDFTFTISSLEAEDAATYYCGQGNRLPYTFGQGTKVEIERTVAAPSVFIFPPSDEQLKSGTASVVCLLNNFYPREAKVQWKVDNALQSGNSQESVTEQDSKDSTYSLSSTLTLSKADYEKHKVYACEVTHQGLSSPVTKSFNRGEC

SEQ ID NO: 184 - protein, 32 aa, synthetic construct; identical to SEQ ID NO: 128
  REGION 1..32: note = An artificially synthesized peptide sequence

SEQ ID NO: 185 - protein, 447 aa, synthetic construct
  REGION 1..447: note = An artificially synthesized peptide sequence
QVQLQESGPGLVRPSQTLSLTCTVSGYSITSDHAWSWVRQPPGRGLEWIGYISYSGITTYNPSLKSRVTMLRDTSKNQFSLRLSSVTAADTAVYYCARSLARTTAMDYWGQGSLVTVSSASTKGPSVFPLAPSSKSTSGGTAALGCLVKDYFPEPVTVSWNSGALTSGVHTFPAVLQSSGLYSLSSVVTVPSSSLGTQTYICNVNHKPSNTKVDKKVEPKSCDKTHTCPPCPAPELLGGPSVFLFPPKPKDTLMISRTPEVTCVVVDVSHEDPEVKFNWYVDGVEVHNAKTKPREEQYNSTYRVVSVLTVLHQDWLNGKEYKCKVSNKALPAPIEKTISKAKGQPREPQVYTLPPSRDELTKNQVSLTCLVKGFYPSDIAVEWESNGQPENNYKTTPPVLDSDGSFFLYSKLTVDKSRWQQGNVFSCSVMHEALHAHYTQKSLSLSP

SEQ ID NO: 186 - protein, 30 aa, synthetic construct
  REGION 1..30: note = An artificially synthesized peptide sequence
QVQLQESGPGLVKPSETLSLTCAVSGHSIS

SEQ ID NO: 187 - protein, 445 aa, synthetic construct
  REGION 1..445: note = An artificially synthesized peptide sequence
QVQLQESGPGLVRPSQTLSLTCTVSGYSITSDHAWSWVRQPPGRGLEWIGYISYSGITTYNPSLKSRVTMLRDTSKNQFSLRLSSVTAADTAVYYCARSLARTTAMDYWGQGSLVTVSSASTKGPSVFPLAPSSKSTSGGTAALGCLVKDYFPEPVTVSWNSGALTSGVHTFPAVLQSSGLYSLSSVVTVPSSNFGTQTYTCNVDHKPSNTKVDKTVERKSCVECPPCPAPPVAGPSVFLFPPKPKDTLMISRTPEVTCVVVDVSHEDPEVQFNWYVDGVEVHNAKTKPREEQFNSTFRVVSVLTVVHQDWLNGKEYKCKVSNKGLPSSIEKTISKAKGQPREPQVYTLPPSREEMTKNQVSLTCLVKGFYPSDIAVEWESNGQPENNYKTTPPMLDSDGSFFLYSKLTVDKSRWQQGNVFSCSVMHEALHNHYTQKSLSLSPGK

SEQ ID NO: 188 - protein, 443 aa, synthetic construct
  REGION 1..443: note = An artificially synthesized peptide sequence
QVQLQESGPGLVRPSQTLSLTCTVSGYSITSDHAWSWVRQPPGRGLEWIGYISYSGITTYNPSLKSRVTMLRDTSKNQFSLRLSSVTAADTAVYYCARSLARTTAMDYWGQGSLVTVSSASTKGPSVFPLAPSSKSTSGGTAALGCLVKDYFPEPVTVSWNSGALTSGVHTFPAVLQSSGLYSLSSVVTVPSSNFGTQTYTCNVDHKPSNTKVDKTVERKSCVECPPCPAPPVAGPSVFLFPPKPKDTLMISRTPEVTCVVVDVSHEDPEVQFNWYVDGVEVHNAKTKPREEQFNSTFRVVSVLTVVHQDWLNGKEYKCKVSNKGLPSSIEKTISKAKGQPREPQVYTLPPSREEMTKNQVSLTCLVKGFYPSDIAVEWESNGQPENNYKTTPPMLDSDGSFFLYSKLTVDKSRWQQGNVFSCSVMHEALHNHYTQKSLSLSP

SEQ ID NO: 189 - protein, 445 aa, synthetic construct
  REGION 1..445: note = An artificially synthesized peptide sequence
QVQLQESGPGLVRPSQTLSLTCTVSGYSITSDHAWSWVRQPPGRGLEWIGYISYSGITTYNPSLKSRVTMLRDTSKNQFSLRLSSVTAADTAVYYCARSLARTTAMDYWGQGSLVTVSSASTKGPSVFPLAPSSKSTSGGTAALGCLVKDYFPEPVTVSWNSGALTSGVHTFPAVLQSSGLYSLSSVVTVPSSNFGTQTYTCNVDHKPSNTKVDKTVERKSCVECPPCPAPPVAGPSVFLFPPKPKDTLMISRTPEVTCVVVDVSHEDPEVQFNWYVDGVEVHNAKTKPREEQFNSTFRVVSVLTVVHQDWLNGKEYKCKVSNKGLPAPIEKTISKTKGQPREPQVYTLPPSREEMTKNQVSLTCLVKGFYPSDIAVEWESNGQPENNYKTTPPMLDSDGSFFLYSKLTVDKSRWQQGNVFSCSVMHEALHNHYTQKSLSLSPGK

SEQ ID NO: 190 - protein, 443 aa, synthetic construct
  REGION 1..443: note = An artificially synthesized peptide sequence
QVQLQESGPGLVRPSQTLSLTCTVSGYSITSDHAWSWVRQPPGRGLEWIGYISYSGITTYNPSLKSRVTMLRDTSKNQFSLRLSSVTAADTAVYYCARSLARTTAMDYWGQGSLVTVSSASTKGPSVFPLAPSSKSTSGGTAALGCLVKDYFPEPVTVSWNSGALTSGVHTFPAVLQSSGLYSLSSVVTVPSSNFGTQTYTCNVDHKPSNTKVDKTVERKSCVECPPCPAPPVAGPSVFLFPPKPKDTLMISRTPEVTCVVVDVSHEDPEVQFNWYVDGVEVHNAKTKPREEQFNSTFRVVSVLTVVHQDWLNGKEYKCKVSNKGLPAPIEKTISKTKGQPREPQVYTLPPSREEMTKNQVSLTCLVKGFYPSDIAVEWESNGQPENNYKTTPPMLDSDGSFFLYSKLTVDKSRWQQGNVFSCSVMHEALHNHYTQKSLSLSP

SEQ ID NO: 191 - protein, 326 aa, synthetic construct
  REGION 1..326: note = An artificially synthesized peptide sequence
ASTKGPSVFPLAPSSKSTSGGTAALGCLVKDYFPEPVTVSWNSGALTSGVHTFPAVLQSSGLYSLSSVVTVPSSNFGTQTYTCNVDHKPSNTKVDKTVERKSCVECPPCPAPPVAGPSVFLFPPKPKDTLMISRTPEVTCVVVDVSHEDPEVQFNWYVDGVEVHNAKTKPREEQFNSTFRVVSVLTVVHQDWLNGKEYKCKVSNKGLPSSIEKTISKAKGQPREPQVYTLPPSREEMTKNQVSLTCLVKGFYPSDIAVEWESNGQPENNYKTTPPMLDSDGSFFLYSKLTVDKSRWQQGNVFSCSVMHEALHNHYTQKSLSLSPGK

SEQ ID NO: 192 - protein, 324 aa, synthetic construct
  REGION 1..324: note = An artificially synthesized peptide sequence
ASTKGPSVFPLAPSSKSTSGGTAALGCLVKDYFPEPVTVSWNSGALTSGVHTFPAVLQSSGLYSLSSVVTVPSSNFGTQTYTCNVDHKPSNTKVDKTVERKSCVECPPCPAPPVAGPSVFLFPPKPKDTLMISRTPEVTCVVVDVSHEDPEVQFNWYVDGVEVHNAKTKPREEQFNSTFRVVSVLTVVHQDWLNGKEYKCKVSNKGLPSSIEKTISKAKGQPREPQVYTLPPSREEMTKNQVSLTCLVKGFYPSDIAVEWESNGQPENNYKTTPPMLDSDGSFFLYSKLTVDKSRWQQGNVFSCSVMHEALHNHYTQKSLSLSP

SEQ ID NO: 193 - protein, 326 aa, synthetic construct
  REGION 1..326: note = An artificially synthesized peptide sequence
ASTKGPSVFPLAPSSKSTSGGTAALGCLVKDYFPEPVTVSWNSGALTSGVHTFPAVLQSSGLYSLSSVVTVPSSNFGTQTYTCNVDHKPSNTKVDKTVERKSCVECPPCPAPPVAGPSVFLFPPKPKDTLMISRTPEVTCVVVDVSHEDPEVQFNWYVDGVEVHNAKTKPREEQFNSTFRVVSVLTVVHQDWLNGKEYKCKVSNKGLPAPIEKTISKTKGQPREPQVYTLPPSREEMTKNQVSLTCLVKGFYPSDIAVEWESNGQPENNYKTTPPMLDSDGSFFLYSKLTVDKSRWQQGNVFSCSVMHEALHNHYTQKSLSLSPGK

SEQ ID NO: 194 - protein, 324 aa, synthetic construct
  REGION 1..324: note = An artificially synthesized peptide sequence
ASTKGPSVFPLAPSSKSTSGGTAALGCLVKDYFPEPVTVSWNSGALTSGVHTFPAVLQSSGLYSLSSVVTVPSSNFGTQTYTCNVDHKPSNTKVDKTVERKSCVECPPCPAPPVAGPSVFLFPPKPKDTLMISRTPEVTCVVVDVSHEDPEVQFNWYVDGVEVHNAKTKPREEQFNSTFRVVSVLTVVHQDWLNGKEYKCKVSNKGLPAPIEKTISKTKGQPREPQVYTLPPSREEMTKNQVSLTCLVKGFYPSDIAVEWESNGQPENNYKTTPPMLDSDGSFFLYSKLTVDKSRWQQGNVFSCSVMHEALHNHYTQKSLSLSP

SEQ ID NO: 195 - protein, 115 aa, synthetic construct
  REGION 1..115: note = Humanized antibody H chain
QVQLVQSGAEVKKPGASVKVSCKASGYTFTDYEMHWVRQAPGQGLEWMGALDPKTGDTAYSQKFKGRVTLTADKSTSTAYMELSSLTSEDTAVYYCTRFYSYTYWGQGTLVTVSS

SEQ ID NO: 196 - protein, 115 aa, synthetic construct
  REGION 1..115: note = Humanized antibody H chain
QVQLVQSGAEVKKPGASVKVSCKASGYTFTDYEMHWIRQPPGQGLEWIGAIDPKTGDTAYSQKFKGRVTLTADKSTSTAYMELSSLTSEDTAVYYCTRFYSYTYWGQGTLVTVSS

SEQ ID NO: 197 - protein, 115 aa, synthetic construct
  REGION 1..115: note = Humanized antibody H chain
QVQLVQSGAEVKKPGASVTVSCKASGYTFTDYEMHWVRQAPGEGLEWMGALDPKTGDTAYSQSFQDRVTLTADKSTSTAYMELSSLTSEDTAVYYCTRFYSYTYWGQGTLVTVSS

SEQ ID NO: 198 - protein, 115 aa, synthetic construct
  REGION 1..115: note = Humanized antibody H chain
QVQLVQSGAEVKKPGASVKVSCKASGYTFTDYEMHWVRQAPGKGLEWMGALNPKTGDTAYSQKFKGRVTLTADKSTSTAYMELSSLTSEDTAVYYCTRFYSYTYWGRGTLVTVSS

SEQ ID NO: 199 - protein, 115 aa, synthetic construct
  REGION 1..115: note = Humanized antibody H chain
QVQLVQSGAEVKKPGASVTVSCKASGYTFTDYEMHWIRQPPGEGLEWIGAIDPKTGDTAYSQSFQDRVTLTADKSTSTAYMELSSLTSEDTAVYYCTRFYSYTYWGQGTLVTVSS

SEQ ID NO: 200 - protein, 115 aa, synthetic construct
  REGION 1..115: note = Humanized antibody H chain
QVQLVQSGAEVKKPGASVKVSCKASGYTFTDYEMHWIRQPPGKGLEWIGAINPKTGDTAYSQKFKGRVTLTADKSTSTAYMELSSLTSEDTAVYYCTRFYSYTYWGRGTLVTVSS

SEQ ID NO: 201 - protein, 112 aa, synthetic construct
  REGION 1..112: note = Humanized antibody L chain
DVVMTQSPLSLPVTPGEPASISCRSSQSLVHSNRNTYLHWYLQKPGQSPQLLIYKVSNRFSGVPDRFSGSGSGTDFTLKISRVEAEDVGVYYCSQNTHVPPTFGQGTKLEIK

SEQ ID NO: 202 - protein, 112 aa, synthetic construct
  REGION 1..112: note = Humanized antibody L chain
DIVMTQSPLSLPVTPGEPASISCRSSQSLVHSNRNTYLHWYQQKPGQAPRLLIYKVSNRFSGVPDRFSGSGSGTDFTLKISRVEAEDVGVYYCSQNTHVPPTFGQGTKLEIK

SEQ ID NO: 203 - protein, 112 aa, synthetic construct
  REGION 1..112: note = Humanized antibody L chain
DVVMTQSPLSLPVTPGEPASISCRASESLVHSNRNTYLHWYLQKPGQSPQLLIYKVSNRFSGVPDRFSGSGSGTDFTLTISSLQAEDVGVYYCSQNTHVPPTFGQGTKLEIK

SEQ ID NO: 204 - protein, 112 aa, synthetic construct
  REGION 1..112: note = Humanized antibody L chain
DVVMTQSPLSLPVTPGQPASISCRASRSLVHSNRNTYLHWYLQKPGQSPQLLIYKVSNRFSGVPDRFSGSGSGTDFTLKISRVEAEDVGVYYCSQNTHVPPTFGRGTKLEIK

SEQ ID NO: 205 - protein, 112 aa, synthetic construct
  REGION 1..112: note = Humanized antibody L chain
DIVMTQSPLSLPVTPGEPASISCRASESLVHSNRNTYLHWYQQKPGQAPRLLIYKVSNRFSGVPDRFSGSGSGTDFTLTISSLQAEDVGVYYCSQNTHVPPTFGQGTKLEIK

SEQ ID NO: 206 - protein, 112 aa, synthetic construct
  REGION 1..112: note = Humanized antibody L chain
DIVMTQSPLSLPVTPGQPASISCRASRSLVHSNRNTYLHWYQQKPGQAPRLLIYKVSNRFSGVPDRFSGSGSGTDFTLKISRVEAEDVGVYYCSQNTHVPPTFGRGTKLEIK

SEQ ID NO: 207 - protein, 545 aa, Homo sapiens
QPPPPPPDATCHQVRSFFQRLQPGLKWVPETPVPGSDLQVCLPKGPTCCSRKMEEKYQLTARLNMEQLLQSASMELKFLIIQNAAVFQEAFEIVVRHAKNYTNAMFKNNYPSLTPQAFEFVGEFFTDVSLYILGSDINVDDMVNELFDSLFPVIYTQLMNPGLPDSALDINECLRGARRDLKVFGNFPKLIMTQVSKSLQVTRIFLQALNLGIEVINTTDHLKFSKDCGRMLTRMWYCSYCQGLMMVKPCGGYCNVVMQGCMAGVVEIDKYWREYILSLEELVNGMYRIYDMENVLLGLFSTIHDSIQYVQKNAGKLTTTIGKLCAHSQQRQYRSAYYPEDLFIDKKVLKVAHVEHEETLSSRRRELIQKLKSFISFYSALPGYICSHSPVAENDTLCWNGQELVERYSQKAARNGMKNQFNLHELKMKGPEPVVSQIIDKLKHINQLLRTMSMPKGRVLDKNLDEEGFEAGDCGDDEDECIGGAGDGMIKVKNQLRFLAELAYDLDVDDAPGNSQQATPKDNEISTFHNLGNVHSPLKHHHHHH

SEQ ID NO: 208 - DNA, 32 bp, synthetic construct
  misc_feature 1..32: note = An artificially synthesized primer sequence
  source 1..32: mol_type = other DNA
ggatcctgcgcatgaaaaagcctgaactcacc

SEQ ID NO: 209 - DNA, 29 bp, synthetic construct
  misc_feature 1..29: note = An artificially synthesized primer sequence
  source 1..29: mol_type = other DNA
gcggccgcctattcctttgccctcggacg

SEQ ID NO: 210 - DNA, 10939 bp, Cricetulus griseus
  source 1..10939: mol_type = unassigned DNA
gagctcaattaaccctcactaaagggagtcgactcgatcctttacagaaaacttgcaaaccctcttggagtagaaaagtagtagtatctgacacaagtatcagcaaaatgcaaacttctccccatccccagaaaaccattataaaaacccccatatcttatgcccaactgtagtgatatattatttatgatttattaaaacttgcttaaggattcagaaagcaaagtcagccttaagctatagagaccaggcagtcagtggtggtacacacctttaatcccaggactcaggattaagaagtagacggacctctgttagttcaagtctaccattacctacacaagagtgaagagtaaccgatctcatgcctttgatcccagcagctgggatcatgtgcattcaatcccagcattcgggagttatataagacaggagcaaggtctcagagctggcattcattctccagccacattgaggataggaaaacattgaagtgtcaggatgctgaggagaggcagcagtttgaggtttggtagaaccaggatcaccttttggtctgaggtagagtaagaactgtggctggctgctttgcttttctgatcttcagcttgaagcttgaactccaatatttgtctctgggtctattattatcatgttacacctaactttaaagctgatttacgcaagacagttgtaggtggacctttctttcctgcccaccagttcccaaataactgacacggagactcaatattaattataaatgattggttaatagctcagtcttgttactggctaactcttacattttaaattaactcatttccatccctttacttgctgccatgtggttcatggcttgttcaagtcctgcttcttctgtctctggctggtgatgcctctggttctgccctttatcccagaattctcctagtctggctctcctgcccagctataggccagtcagctgtttattaaccaatgagaataatacatatttatagtgtacaaagattgctcctcaacacccaattttttatgtgcaacctgagaatctggactcattgccctcatgcttgcagaggcggcacccttacccactaagccacctttctagccctgttgcttttgttttttgagacaggttccactatgtagcccaggctggcctcaaactgaccattctcctgcctaaacctcccgaacactggaattatagtcaaggcctacctgccctggcattttcacacttttatttcctggctgagtccattgactttacactcatcaaggttgaaccagttggagtttaattacagtgccaatcgcactgaatcccacataatcaaacaacttcaaggaagcaaaaaaccagtttttcctgaagatcaatgtcagcttgcctgattcagaatagacccccgaaaaaaggcaaatgcttgataaccaatttcttcttattgttcaatcccctgctgctgtgtgtaagctcctgagaaaggacagtaaggggacattcatgatcagagaaagagccccaactccccccccagccccacccccaccctgtccacagtctgttggtttggtttccccctggctgacacccagaaatcacaacataatcacctaggtcactgtaacaagttcctttctggaaaatgctacaaatgatattggtaacatgagtaatgaataatgcctggagtccaactcccttgtgacccagcaatgttttccgtgggtgctcccttccccagctgcaggcctgacatgtaccttaaaaagcctcccctggaggacagaattttgtgggtactatagtgttctcacaaatacttcccctaatacccttacttagttaccataaataacatgcagcccctggtgaggcacacagggctccaatgtacagcttctcagacactgcaggaaccttcctctcctaatgcagcactggtctcttcaggctggacagcaggaacccataccactccaatcctagtgtggagtagagctgtctacgaaaaccagcagatctatagctaaatgtgtttcaattttatgctttgacaaattgtactgaccccacccccaccccttcccccttgctgtgctgggaattgaacccaggaccttgtgcatgccaggcaagtactctaacactgagctatagccccaatctttcatccaagtctctatgtgtgcccacactcgctttttattttgagacaaaaggttcttattttgagataaggtctcactatgttgccttgacttttttttttttttttttttgaacttttgaccttcctacctcagctgagactacaagtcttttaccatcaggcccggctgatggtaaaataacagtatttgaaatagtttaaacacatcatcttaatggtcaaccacacaatttccgaaatgttgctggctcagtctggggcaaacctgtccgccccaacattggtgctaggaagaaagcacagacaagtagccctcccagctcaggagtaaaagacctggagggggtggcccacttcggtcaagttcacgggatggggaggggtaccctcctccagtagtggtggtatttggcagttcctccaccgacgccctctggaagcacctgcttggacccgcaaagccaggaatgcagcttcctcaagggactcgccagcgagggtaacaggacagaggcgtcccaagagggctggggcggaagggggaagacagggtcggccttagatagggcaaagggccttctggctgtgttcccggggtaaccgccccaccacgcctggagcccgacgtggcgagcgatggggacagcgagcaggaagtcgtactggggagggccgcgtagcagatgcagccgagggcggcgctgccaggtacacccgagggcaccgcgggggtgagcgccaggtccctgaaccagccaggcctccagagccgagtccggcggaccgacggtacgttctggaatgggaagggatccgggacaccgaattgctgcattgaggggctcagaggttctgatgtgggagtccagaaagggttttatctaccggaggtgatgtgacttccggcctctggaagtgctgttggagtctctgggaccttgggtcctctcgactaggtttggaaggggtgaaataggggtagggagaaaggagaggactgcagcaatgtcttcccgaacgacctgggttcgggaggggtcgaaggacaaggggctgttgtggggggtcttcagacgcggaggggtggtattctattttctgggaagatggtgtcgatgcacttgaccaagtctagtcgatctgaagaggctaggggaacagacagtgagagaggatggtggagggagtggcagaacccttccagaaactgggagaggctctagcacctgcaaccccttccctggcctccggggagtcccagaagagggcaggaccatggacacaggtgcattcgtgccggcgcgctccggcctggcgaaggtgcgcgctcttggaggccgcgggagggccagacgcgcgcccggagagctggccctttaaggctacccggaggcgtgtcaggaaatgcgccctgagcccgcccctcccggaacgcggcccgagacctggcaagctgagacggaactcggaactagcactcggctcgcggcctcggtgaggccttgcgcccgccatgcctctgtcattgcccctcgggccgcctccctgaacctccgtgaccgccctgcagtcctccctcccccccttcgactcggcgggcgcttccgggcgctcccgcagcccgccctccacgtagcccacacctccctctcggcgctccgcttcccacgcggtccccgacctgttctttcctcctccaccctgcccttctgtccctctcccttcctttctcccctcgactcgtccctattaggcaacagcccctgtggtccagccggccatggctgtcaaggctcacacccttagctaggccccttctcccttccctgggtcttgtctcatgaccccctgccccgcccgggagcgagcgcgatgtggagcagtgcctctggcaagcagaacttcacccaagccatgtgacaattgaaggctgtacccccagaccctaacatcttggagccctgtagaccagggagtgcttctggccgtggggtgacctagctcttctaccaccatgaacagggcccctctgaagcggtccaggatcctgcgcatggcgctgactggaggctccactgcctctgaggaggcagatgaagacagcaggaacaagccgtttctgctgcgggcgctgcagatcgcgctggtcgtctctctctactgggtcacctccatctccatggtattcctcaacaagtacctgctggacagcccctccctgcagctggatacccctatcttcgtcactttctaccaatgcctggtgacctctctgctgtgcaagggcctcagcactctggccacctgctgccctggcaccgttgacttccccaccctgaacctggaccttaaggtggcccgcagcgtgctgccactgtcggtagtcttcattggcatgataagtttcaataacctctgcctcaagtacgtaggggtggccttctacaacgtggggcgctcgctcaccaccgtgttcaatgtgcttctgtcctacctgctgctcaaacagaccacttccttctatgccctgctcacatgtggcatcatcattggtgagtggggcccgggggctgtgggagcaggatgggcatcgaactgaagccctaaaggtcaacactgtaggtacctttacttactgtcccaggtcccttgcatcagcagttacaggaagagccctgtagaaaacaaataacttccttatggtcattcaacaagttagggacccagccagggtgaaaataatgttagcagcaactacagcaaagatggctctcgccacttgcatgattaaaatgtgccaggtactcagatctaagcattggatccacattaactcaactaatccctattacaaggtaaaatatatccgaattttacagagggaaaaccaaggcacagagaggctaagtagcttgaccaggatcacacagctaataatcactgacatagctgggatttaaacataagcagttacctccatagatcacactatgaccaccatgccactgttccttctcaagagttccaggatcctgtctgtccagttctctttaaagaggacaacacatctgacattgctaccttgaggtaacatttgaaatagtgggtagacatatgttttaagttttattcttactttttatgtgtgtgtgtttggggggccaccacagtgtatgggtggagataaggggacaacttaagaattggtcctttctcccaccacatgggtgctgaggtctgaactcaggtcatcaggattggcacaaatccctttacccactgagccatttcactggtccaatatatgtgtgcttttaagaggctttaactattttcccagatgtgaatgtcctgctgatcattatccccttttacccggaagccctctgggaggtgccatccctgtggtcgtctgcatacaaatggggaaactgcaactcagagaaacaaggctacttgccagggccccacaagtaagataggctgggatgccatcccagactggccacactccctggcctgtgcttcaagccagtttactttgttcctgcccattggaagttagcatgttgcagtcaaacacaataactacaggccaaaagtgcttttaaattaaagtcagatgaacttttaaacatccagagctcctcaactgcaggagttacaacctgattctgcaaccatctttgcagtgcccggtagtcatatgtagctagaggctcttggctaggacagcatgtgttaggaaacatctggccctgagatcattgaattgagtgactgctgggtgacaaagaccaaggcatccgttccctgagagtcctgggcaagcagcaatgtgaccttcatttgtacctactcaggttctttatctgtcctgtttgacctacttagtctcctctggtgtctcagaggcccaggctgggtactctggatgtcaggatcaggccaatgcgcacatctgccctagaaatgtccccctggttgagcagctcctgaatccatcggtaaagggtctggaccagggaggagtcagataaaaagctgacagcactgggggactccatggggaactcccacctgcccccacacatccatcctaagagaactggtattccttgtttcctctttgtcctacaaggcaccctgggatcccacttcagtctcccagccttgccagggttagagggcatgagcctccttgtggggaatttagatgcaagaaggtacagtcactagagaacctgagctcagatccccaaagtaaccagtacctgatagtgaggcagctgagaaccgcagcagcctgcctgagtggctgaactctgcggcctccggaactggccccaactgttgggtctcctcttccttcctcctgtgagggagggcccatctctgataagtgctgtggggactctagagtagggaggaggaggagcaatctaagcaggccttactgagaagtccttgctggcatgtggctgcctgaggagtacagactgggaacacccatttgaatgagtaaggtttttcctgaaggccatggggagccacggaggaaaatcattttagttacaagacaaagagtagattggttaacatgggagcaaggacatggccccaattttcatagatgaaggaaattggaactcagagaggttaagtaacttctcccaaatagctcagcttcaaaatcacagaacagtcagagtctagatctctctgatgcctgtgatggtcctgccattccatgttgctgatccctgtggcatcagtaagcctctaccttgtgggaatgcaggatctaaatgaagagaggaagtgctggccccatgctgtggtctggaaagctatgcaggctctttgagcagagagtgacccacaagtgaatagagtcctatgagactcaaagcaacatccacccttaagcagctctaaccaaatgctcacactgagggagccaaagccaagttagagtcctgtgcttgcccaaggtcactttgcctggccctcctcctatagcacccgtgttatcttatagccctcattacagtgattacaattataattagagaggtaacagggccacactgtccttacacattcccctgctagattgtagctgggagagggggagatgtaggtggctgggggagtgggagggaagatgcagattttcattctgggctctactccctcagccattttttggtgtgggagttagactttggatatgttgatgatgaggtaagggccacagaacagtctgaactgtggtatcagaatcctgtccctctccctctctcctcatccctcttcaccttgtcactcctctgtctgctacaggtggtttctggctgggtatagaccaagagggagctgagggcaccctgtccctcataggcaccatcttcggggtgctggccagcctctgcgtctccctcaatgccatctataccaagaaggtgctcccagcagtggacaacagcatctggcgcctaaccttctataacaatgtcaatgcctgtgtgctcttcttgcccctgatggttctgctgggtgagctccgtgccctccttgactttgctcatctgtacagtgcccacttctggctcatgatgacgctgggtggcctcttcggctttgccattggctatgtgacaggactgcagatcaaattcaccagtcccctgacccacaatgtatcaggcacagccaaggcctgtgcgcagacagtgctggccgtgctctactatgaagagactaagagcttcctgtggtggacaagcaacctgatggtgctgggtggctcctcagcctatacctgggtcaggggctgggagatgcagaagacccaagaggaccccagctccaaagagggtgagaagagtgctattggggtgtgagcttcttcagggacctgggactgaacccaagtggggcctacacagcactgaaggcttcccatggagctagccagtgtggccctgagcaatactgtttacatcctccttggaatatgatctaagaggagccagggtctttcctggtaatgtcagaaagctgccaaatctcctgtctgccccatcttgttttgggaaaaccctaccaggaatggcacccctacctgcctcctcctagagcctgtctacctccatatcatctctggggttgggaccagctgcagccttaaggggctggattgatgaagtgatgtcttctacacaagggagatgggttgtgatcccactaattgaagggatttgggtgaccccacacctctgggatccagggcaggtagagtagtagcttaggtgctattaacatcaggaacacctcagcctgcctttgaagggaagtgggagcttggccaagggaggaaatggccattctgccctcttcagtgtggatgagtatggcagacctgttcatggcagctgcaccctggggtggctgataagaaaacattcacctctgcatttcatatttgcagctctagaacgggggagagccacacatcttttacgggttaagtagggtgatgagctcctccgcagtccctaaccccagctttacctgcctggcttcccttggcccagctacctagctgtactccctttctgtactcttctcttctccgtcatggcctcccccaacacctccatctgcaggcaggaagtggagtccacttgtaacctctgttcccatgacagagccctttgaatacctgaacccctcatgacagtaagagacatttatgttctctggggctggggctgaaggagcccactggttctcacttagcctatctggctcctgtcacaaaaaaaaaaaaagaaaaaaaaaaagcataaaccaagttactaagaacagaagttggtttataacgttctggggcagcaaagcccagatgaagggacccatcgaccctctctgtccatatcctcatgctgcagaagtacaggcaagctcctttaagcctcatataggaacactagcctcactcatgagggttttactccatgacctgtcaacctcaaagccttcaacatgaggactccaacgtaaatttggggacagaagcactcagaccataccccagcaccacaccctcctaacctcagggtagctgtcattctcctagtctcctctcttgggcctttagaacccccatttccttggggtaatgtctgatgtttttgtccctgtcataaaaagatggagagactgtgtccagcctttgattcctacttcctacaatcccaggttctaatgaagtttgtggggcctgatgccctgagttgtatgtgatttaataataaaaaagcaagatacagcatgtgtgtggactgagtgagggccacagggatctaaaagccaagtgtgaggggacccagctacagcaggcagcatcctgagcctggaatctcttcaggacaagaattctccatatacctacctactctggggagtaggtggccagagttcaagcttcccttagtaccaactaccactggctgtgctcttactgaaggcagacatggcactgagtgctgtccatctgtcactcatctccacagccattcctaatgtgtggggtgggagccatcaccaaaccccattttcagataaggacacaggctcagagaggcttgtgtggagaaaagtagcagcagaattcagagagctgggtctcctgcagcaccttggactgccagcagccacagtgcttgtcacacagcacatactcaaaagaatgccagccccctcagcctagagtgcctggcctttctttcagatgaggaagagggtcaaagctgttagcttgcccaccatatgaccacatacatgaccaacagcttgagggagggaggattactgtggctcccagcctgagaggtgggacacccaaatgtattaggtccttgaatcagggctgaccttgtgattcagtcactcctaccagaatgctggggaatggggatgccaaaggcaaaggaggctttctaaggtgtggtgtaagataggcatttctgcttccatgtacacctgtgagcagagtaggaaggccctgtggagaatatatcccacaaaccagtagcccttcctggcagtgggtgaatactgccaccctatacccctatgcaaggccagtagaaccacccaacccacaacatctagagaaattacaggtcatcttaagcctctaaattgtggagaaactcgacatgcgcacgattcctaacctgctagcctagggtgcggggtggataatttaaggaaactggggtttcttatagaatcggaggctccatgaagtcaccctgacaagaggtcagcaatagccagcagcagtggctactcctaagcctccagacagagcaccctgtgaatgtaccttattctcacatctgggtgtctataggtgtgactgggtcagatgtcacccaggccattgcaatgggcccttagccccatggggtgttgggatagcagccaagcagctcccatgctgagatactgcctgcagtagactgatggataagaaaacaaggcccaaaatgttttctttccagacttgatctttctttgttcaaaaatgctgttttcccttaaacttgcccaaacccattgttttgcagttgaggaaaataaggcatagaaagattaaaggaagtttctgaggttacagagcaaagtactggcttcacctgaaatagacaggtgtgccctgatcctgatttgagctc

SEQ ID NO: 211 - DNA, 33 bp, synthetic construct
  misc_feature 1..33: note = An artificially synthesized primer sequence
  source 1..33: mol_type = other DNA
atgcatgccaccatgaaaaagcctgaactcacc

SEQ ID NO: 212 - DNA, 28 bp, synthetic construct
  misc_feature 1..28: note = An artificially synthesized primer sequence
  source 1..28: mol_type = other DNA
ggatcccaggctttacactttatgcttc

SEQ ID NO: 213 - DNA, 25 bp, synthetic construct
  misc_feature 1..25: note = An artificially synthesized primer sequence
  source 1..25: mol_type = other DNA
gctgtctggagtactgtgcatctgc

SEQ ID NO: 214 - DNA, 27 bp, synthetic construct
  misc_feature 1..27: note = An artificially synthesized primer sequence
  source 1..27: mol_type = other DNA
ggaatgcagcttcctcaagggactcgc

SEQ ID NO: 215 - DNA, 27 bp, synthetic construct
  misc_feature 1..27: note = An artificially synthesized primer sequence
  source 1..27: mol_type = other DNA
tgcatcaggtcggagacgctgtcgaac

SEQ ID NO: 216 - DNA, 27 bp, synthetic construct
  misc_feature 1..27: note = An artificially synthesized primer sequence
  source 1..27: mol_type = other DNA
gcactcgtccgagggcaaaggaatagc

SEQ ID NO: 217 - DNA, 24 bp, synthetic construct
  misc_feature 1..24: note = An artificially synthesized primer sequence
  source 1..24: mol_type = other DNA
tgtgctgggaattgaacccaggac

SEQ ID NO: 218 - DNA, 22 bp, synthetic construct
  misc_feature 1..22: note = An artificially synthesized primer sequence
  source 1..22: mol_type = other DNA
ctacttgtctgtgctttcttcc

SEQ ID NO: 219 - DNA, 27 bp, synthetic construct
  misc_feature 1..27: note = An artificially synthesized primer sequence
  source 1..27: mol_type = other DNA
ctcgactcgtccctattaggcaacagc

SEQ ID NO: 220 - DNA, 27 bp, synthetic construct
  misc_feature 1..27: note = An artificially synthesized primer sequence
  source 1..27: mol_type = other DNA
tcagaggcagtggagcctccagtcagc

SEQ ID NO: 221 - protein, 449 aa, Homo sapiens
QVQLQESGPGLVRPSQTLSLTCTVSGYSITSDHAWSWVRQPPGRGLEWIGYISYSGITTYNPSLKSRVTMLRDTSKNQFSLRLSSVTAADTAVYYCARVLARITAMDYWGQGSLVTVSSASTKGPSVFPLAPSSKSTSGGTAALGCLVKDYFPEPVTVSWNSGALTSGVHTFPAVLQSSGLYSLSSVVTVPSSSLGTQTYICNVNHKPSNTKVDKKVEPKSCDKTHTCPPCPAPELLGGPSVFLFPPKPKDTLMISRTPEVTCVVVDVSHEDPEVKFNWYVDGVEVHNAKTKPREEQYNSTYRVVSVLTVLHQDWLNGKEYKCKVSNKALPAPIEKTISKAKGQPREPQVYTLPPSRDELTKNQVSLTCLVKGFYPSDIAVEWESNGQPENNYKTTPPVLDSDGSFFLYSKLTVDKSRWQQGNVFSCSVMHEALHNHYTQKSLSLSPGK

SEQ ID NO: 222 - protein, 449 aa, synthetic construct
  REGION 1..449: note = An artificially synthesized peptide sequence
QVQLQESGPGLVKPSETLSLTCAVSGYSISDDHAWSWVRQPPGEGLEWIGYISYSGITNYNPSLKGRVTISRDTSKNQFSLKLSSVTAADTAAYYCARVLARITAMDYWGEGTLVTVSSASTKGPSVFPLAPSSKSTSGGTAALGCLVKDYFPEPVTVSWNSGALTSGVHTFPAVLQSSGLYSLSSVVTVPSSSLGTQTYICNVNHKPSNTKVDKKVEPKSCDKTHTCPPCPAPELLGGPSVFLFPPKPKDTLMISRTPEVTCVVVDVSHEDPEVKFNWYVDGVEVHNAKTKPREEQYNSTYRVVSVLTVLHQDWLNGKEYKCKVSNKALPAPIEKTISKAKGQPREPQVYTLPPSRDELTKNQVSLTCLVKGFYPSDIAVEWESNGQPENNYKTTPPVLDSDGSFFLYSKLTVDKSRWQQGNVFSCSVMHEALHNHYTQKSLSLSPGK

SEQ ID NO: 223 - protein, 449 aa, synthetic construct; identical to SEQ ID NO: 135
  REGION 1..449: note = An artificially synthesized peptide sequence

SEQ ID NO: 224 - protein, 214 aa, Homo sapiens
DIQMTQSPSSLSASVGDRVTITCRASQDISSYLNWYQQKPGKAPKLLIYYTSRLHSGVPSRFSGSGSGTDFTFTISSLQPEDIATYYCGQGNRLPYTFGQGTKVEIKRTVAAPSVFIFPPSDEQLKSGTASVVCLLNNFYPREAKVQWKVDNALQSGNSQESVTEQDSKDSTYSLSSTLTLSKADYEKHKVYACEVTHQGLSSPVTKSFNRGEC

SEQ ID NO: 225 - protein, 214 aa, synthetic construct
  REGION 1..214: note = An artificially synthesized peptide sequence
DIQMTQSPSSLSASVGDSVTITCQASQDISSYLNWYQQKPGKAPELLIYYGSELHSGVPSRFSGSGSGTDFTFTISSLEAEDAATYYCGQGNRLPYTFGQGTKVEIERTVAAPSVFIFPPSDEQLKSGTASVVCLLNNFYPREAKVQWKVDNALQSGNSQESVTEQDSKDSTYSLSSTLTLSKADYEKHKVYACEVTHQGLSSPVTKSFNRGEC

SEQ ID NO: 226 - protein, 214 aa, synthetic construct; identical to SEQ ID NO: 136
  REGION 1..214: note = An artificially synthesized peptide sequence

SEQ ID NO: 227 - protein, 449 aa, Homo sapiens
QVQLQESGPGLVRPSQTLSLTCTVSGYSITSDHAWSWVRQPPGRGLEWIGYISYSGITTYNPSLKSRVTMLRDTSKNQFSLRLSSVTAADTAVYYCARSLARTTAMDYWGQGSLVTVSSASTKGPSVFPLAPSSKSTSGGTAALGCLVKDYFPEPVTVSWNSGALTSGVHTFPAVLQSSGLYSLSSVVTVPSSSLGTQTYICNVNHKPSNTKVDKKVEPKSCDKTHTCPPCPAPELLGGPSVFLFPPKPKDTLMISRTPEVTCVVVDVSHEDPEVKFNWYVDGVEVHNAKTKPREEQYNSTYRVVSVLTVLHQDWLNGKEYKCKVSNKALPAPIEKTISKAKGQPREPQVYTLPPSRDELTKNQVSLTCLVKGFYPSDIAVEWESNGQPENNYKTTPPVLDSDGSFFLYSKLTVDKSRWQQGNVFSCSVMHEALHNHYTQKSLSLSPGK

SEQ ID NO: 228 - protein, 449 aa, synthetic construct
  REGION 1..449: note = An artificially synthesized peptide sequence
QVQLQESGPGLVKPSETLSLTCAVSGYSISDDHAWSWVRQPPGEGLEWIGYISYSGITNYNPSLKGRVTISRDTSKNQFSLKLSSVTAADTAAYYCARSLARTTAMDYWGEGTLVTVSSASTKGPSVFPLAPSSKSTSGGTAALGCLVKDYFPEPVTVSWNSGALTSGVHTFPAVLQSSGLYSLSSVVTVPSSSLGTQTYICNVNHKPSNTKVDKKVEPKSCDKTHTCPPCPAPELLGGPSVFLFPPKPKDTLMISRTPEVTCVVVDVSHEDPEVKFNWYVDGVEVHNAKTKPREEQYNSTYRVVSVLTVLHQDWLNGKEYKCKVSNKALPAPIEKTISKAKGQPREPQVYTLPPSRDELTKNQVSLTCLVKGFYPSDIAVEWESNGQPENNYKTTPPVLDSDGSFFLYSKLTVDKSRWQQGNVFSCSVMHEALHNHYTQKSLSLSPGK

SEQ ID NO: 229 - protein, 214 aa, Homo sapiens [sequence omitted]

SEQ ID NO: 230 - protein, 214 aa, synthetic construct
  REGION 1..214: note = An artificially synthesized peptide sequence
DIQMTQSPSSLSASVGDSVTITCQASQDISSYLNWYQQKPGKAPELLIYYGSELHSGVPSRFSGSGSGTDFTFTISSLEAEDAATYYCQQGNSLPYTFGQGTKVEIERTVAAPSVFIFPPSDEQLKSGTASVVCLLNNFYPREAKVQWKVDNALQSGNSQESVTEQDSKDSTYSLSSTLTLSKADYEKHKVYACEVTHQGLSSPVTKSFNRGEC

SEQ ID NO: 231 - protein, 214 aa, synthetic construct
  REGION 1..214: note = An artificially synthesized peptide sequence
DIQMTQSPSSLSASVGDSVTITCQASQDISSYLNWYQQKPGKAPELLIYYGSEEHSGVPSRFSGSGSGTDFTFTISSLEAEDAATYYCQQGNSLPYTFGQGTKVEIERTVAAPSVFIFPPSDEQLKSGTASVVCLLNNFYPREAKVQWKVDNALQSGNSQESVTEQDSKDSTYSLSSTLTLSKADYEKHKVYACEVTHQGLSSPVTKSFNRGEC

SEQ ID NO: 232 - protein, 214 aa, synthetic construct
  REGION 1..214: note = An artificially synthesized peptide sequence
DIQMTQSPSSLSASVGDSVTITCQASQDISSYLNWYQQKPGKAPELLIYYGSELESGVPSRFSGSGSGTDFTFTISSLEAEDAATYYCQQGNSLPYTFGQGTKVEIERTVAAPSVFIFPPSDEQLKSGTASVVCLLNNFYPREAKVQWKVDNALQSGNSQESVTEQDSKDSTYSLSSTLTLSKADYEKHKVYACEVTHQGLSSPVTKSFNRGEC

SEQ ID NO: 233 - protein, 445 aa, Homo sapiens
QVQLVQSGAEVKKPGASVKVSCKASGYTFTDYEMHWIRQPPGKGLEWIGAINPKTGDTAYSQKFKGRVTLTADKSTSTAYMELSSLTSEDTAVYYCTRFYSYTYWGRGTLVTVSSASTKGPSVFPLAPSSKSTSGGTAALGCLVKDYFPEPVTVSWNSGALTSGVHTFPAVLQSSGLYSLSSVVTVPSSSLGTQTYICNVNHKPSNTKVDKKVEPKSCDKTHTCPPCPAPELLGGPSVFLFPPKPKDTLMISRTPEVTCVVVDVSHEDPEVKFNWYVDGVEVHNAKTKPREEQYNSTYRVVSVLTVLHQDWLNGKEYKCKVSNKALPAPIEKTISKAKGQPREPQVYTLPPSRDELTKNQVSLTCLVKGFYPSDIAVEWESNGQPENNYKTTPPVLDSDGSFFLYSKLTVDKSRWQQGNVFSCSVMHEALHNHYTQKSLSLSPGK

SEQ ID NO: 234 - protein, 445 aa, synthetic construct
  REGION 1..445: note = An artificially synthesized peptide sequence
QVQLVQSGAEVKKPGASVKVSCKASGYTFTDYEMHWVRQAPGQGLEWMGALDPKTGDTAYSQKFKGRVTLTADKSTSTAYMELSSLTSEDTAVYYCTRFYSYTYWGQGTLVTVSSASTKGPSVFPLAPSSKSTSGGTAALGCLVKDYFPEPVTVSWNSGALTSGVHTFPAVLQSSGLYSLSSVVTVPSSSLGTQTYICNVNHKPSNTKVDKKVEPKSCDKTHTCPPCPAPELLGGPSVFLFPPKPKDTLMISRTPEVTCVVVDVSHEDPEVKFNWYVDGVEVHNAKTKPREEQYNSTYRVVSVLTVLHQDWLNGKEYKCKVSNKALPAPIEKTISKAKGQPREPQVYTLPPSRDELTKNQVSLTCLVKGFYPSDIAVEWESNGQPENNYKTTPPVLDSDGSFFLYSKLTVDKSRWQQGNVFSCSVMHEALHNHYTQKSLSLSPGK

SEQ ID NO: 235 - protein, 445 aa, synthetic construct
  REGION 1..445: note = An artificially synthesized peptide sequence
QVQLVQSGAEVKKPGASVTVSCKASGYTFTDYEMHWIRQPPGEGLEWIGAIDPKTGDTAYSESFQDRVTLTADKSTSTAYMELSSLTSEDTAVYYCTRFYSYTYWGQGTLVTVSSASTKGPSVFPLAPSSKSTSGGTAALGCLVKDYFPEPVTVSWNSGALTSGVHTFPAVLQSSGLYSLSSVVTVPSSSLGTQTYICNVNHKPSNTKVDKKVEPKSCDKTHTCPPCPAPELLGGPSVFLFPPKPKDTLMISRTPEVTCVVVDVSHEDPEVKFNWYVDGVEVHNAKTKPREEQYNSTYRVVSVLTVLHQDWLNGKEYKCKVSNKALPAPIEKTISKAKGQPREPQVYTLPPSRDELTKNQVSLTCLVKGFYPSDIAVEWESNGQPENNYKTTPPVLDSDGSFFLYSKLTVDKSRWQQGNVFSCSVMHEALHNHYTQKSLSLSPGK

SEQ ID NO: 236 - protein, 219 aa, Homo sapiens
DIVMTQSPLSLPVTPGQPASISCRASRSLVHSNRNTYLHWYQQKPGQAPRLLIYKVSNRFSGVPDRFSGSGSGTDFTLKISRVEAEDVGVYYCSQNTHVPPTFGRGTKLEIKRTVAAPSVFIFPPSDEQLKSGTASVVCLLNNFYPREAKVQWKVDNALQSGNSQESVTEQDSKDSTYSLSSTLTLSKADYEKHKVYACEVTHQGLSSPVTKSFNRGEC

SEQ ID NO: 237 - protein, 219 aa, synthetic construct
  REGION 1..219: note = An artificially synthesized peptide sequence
DVVMTQSPLSLPVTPGEPASISCRSSQSLVHSNRNTYLHWYLQKPGQSPQLLIYKVSNRFSGVPDRFSGSGSGTDFTLKISRVEAEDVGVYYCSQNTHVPPTFGQGTKLEIKRTVAAPSVFIFPPSDEQLKSGTASVVCLLNNFYPREAKVQWKVDNALQSGNSQESVTEQDSKDSTYSLSSTLTLSKADYEKHKVYACEVTHQGLSSPVTKSFNRGEC

SEQ ID NO: 238 - protein, 219 aa, synthetic construct
  REGION 1..219: note = An artificially synthesized peptide sequence
DIVMTQSPLSLPVTPGEPASISCQASESLVHSNRNTYLHWYLQKPGQSPQLLIYKVSNRFSGVPDRFSGSGSGTDFTLKISRVEAEDVGVYYCSQNTHVPPTFGQGTKVEIERTVAAPSVFIFPPSDEQLKSGTASVVCLLNNFYPREAKVQWKVDNALQSGNSQESVTEQDSKDSTYSLSSTLTLSKADYEKHKVYACEVTHQGLSSPVTKSFNRGEC

SEQ ID NO: 239 - protein, 447 aa, Homo sapiens
QVQLVQSGAEVKKPGASVKVSCKASGYTFTGYIMNWVRQAPGQGLEWMGLINPYNGGTSYNQKFKGRVTITADESTSTAYMELSSLRSEDTAVYYCARDGYDDGPYTMDYWGQGTLVTVSSASTKGPSVFPLAPSSKSTSESTAALGCLVKDYFPEPVTVSWNSGALTSGVHTFPAVLQSSGLYSLSSVVTVPSSNFGTQTYTCNVDHKPSNTKVDKTVERKSCVECPPCPAPPVAGPSVFLFPPKPKDTLMISRTPEVTCVVVDVSHEDPEVQFNWYVDGVEVHNAKTKPREEQFNSTFRVVSVLTVVHQDWLNGKEYKCKVSNKGLPAPIEKTISKTKGQPREPQVYTLPPSREEMTKNQVSLTCLVKGFYPSDIAVEWESNGQPENNYKTTPPMLDSDGSFFLYSKLTVDKSRWQQGNVFSCSVMHEALHNHYTQKSLSLSPGK

SEQ ID NO: 240 - protein, 447 aa, synthetic construct
  REGION 1..447: note = An artificially synthesized peptide sequence
QVQLVQSGAEVKKPGASVKVSCKASGYTFTGYIMNWVRQAPGQGLEWMGLINPYNGGTSYNQQFQDRVTITADESTSTAYMELSSLRSEDTAVYYCARDGYDDGPYTMDYWGQGTLVTVSSASTKGPSVFPLAPSSKSTSESTAALGCLVKDYFPEPVTVSWNSGALTSGVHTFPAVLQSSGLYSLSSVVTVPSSNFGTQTYTCNVDHKPSNTKVDKTVERKSCVECPPCPAPPVAGPSVFLFPPKPKDTLMISRTPEVTCVVVDVSHEDPEVQFNWYVDGVEVHNAKTKPREEQFNSTFRVVSVLTVVHQDWLNGKEYKCKVSNKGLPAPIEKTISKTKGQPREPQVYTLPPSREEMTKNQVSLTCLVKGFYPSDIAVEWESNGQPENNYKTTPPMLDSDGSFFLYSKLTVDKSRWQQGNVFSCSVMHEALHNHYTQKSLSLSPGK

SEQ ID NO: 241 - protein, 447 aa, synthetic construct
  REGION 1..447: note = An artificially synthesized peptide sequence
QVQLVQSGAEVKKPGASVKVSCKASGYTFTGYIMNWVRQAPGQGLEWMGLINPYNGGTSYNDQFQDRVTITADESTSTAYMELSSLRSEDTAVYYCARDGYDDGPYTMDYWGQGTLVTVSSASTKGPSVFPLAPSSKSTSESTAALGCLVKDYFPEPVTVSWNSGALTSGVHTFPAVLQSSGLYSLSSVVTVPSSNFGTQTYTCNVDHKPSNTKVDKTVERKSCVECPPCPAPPVAGPSVFLFPPKPKDTLMISRTPEVTCVVVDVSHEDPEVQFNWYVDGVEVHNAKTKPREEQFNSTFRVVSVLTVVHQDWLNGKEYKCKVSNKGLPAPIEKTISKTKGQPREPQVYTLPPSREEMTKNQVSLTCLVKGFYPSDIAVEWESNGQPENNYKTTPPMLDSDGSFFLYSKLTVDKSRWQQGNVFSCSVMHEALHNHYTQKSLSLSPGK

SEQ ID NO: 242 - protein, 214 aa, Homo sapiens
DIQMTQSPSSLSASVGDRVTITCRTSENIYSFLAWYQQKPGKAPKLLIYNAKTLAKGVPSRFSGSGSGTDFTLTISSLQPEDFATYYCQHHYESPLTFGGGTKVEIKRTVAAPSVFIFPPSDEQLKSGTASVVCLLNNFYPREAKVQWKVDNALQSGNSQESVTEQDSKDSTYSLSSTLTLSKADYEKHKVYACEVTHQGLSSPVTKSFNRGEC

SEQ ID NO: 243 - protein, 214 aa, synthetic construct
  REGION 1..214: note = An artificially synthesized peptide sequence
DIQMTQSPSSLSASVGDRVTITCQTSEDIYSFLAWYQQKPGKAPKLLIYNAQTEAQGVPSRFSGSGSGTDFTLTISSLQPEDFATYYCQHHYESPLTFGGGTKVEIKRTVAAPSVFIFPPSDEQLKSGTASVVCLLNNFYPREAKVQWKVDNALQSGNSQESVTEQDSKDSTYSLSSTLTLSKADYEKHKVYACEVTHQGLSSPVTKSFNRGEC

SEQ ID NO: 244 - protein, 445 aa, synthetic construct
  REGION 1..445: note = An artificially synthesized peptide sequence
QVQLVQSGAEVKKPGASVKVSCKASGYTFTGYIMNWVRQAPGQGLEWMGLINPYNGGTSYNQKFKGRVTITADESTSTAYMELSSLRSEDTAVYYCARDGYDDGPYTMDYWGQGTLVTVSSASTKGPSVFPLAPSSKSTSGGTAALGCLVKDYFPEPVTVSWNSGALTSGVHTFPAVLQSSGLYSLSSVVTVPSSNFGTQTYTCNVDHKPSNTKVDKTVERKSCVECPPCPAPPVAGPSVFLFPPKPKDTLMISRTPEVTCVVVDVSQEDPEVQFNWYVDGVEVHNAKTKPREEQFNSTFRVVSVLTVVHQDWLNGKEYKCKVSNKGLPAPIEKTISKTKGQPREPQVYTLPPSQEEMTKNQVSLTCLVKGFYPSDIAVEWESNGQPENNYKTTPPMLDSDGSFFLYSKLTVDKSRWQEGNVFSCSVMHEALHNHYTQKSLSLSP

SEQ ID NO: 245 - protein, 445 aa, synthetic construct
  REGION 1..445: note = An artificially synthesized peptide sequence
QVQLVQSGAEVKKPGASVKVSCKASGYTFTGYIMNWVRQAPGQGLEWMGLINPYNGGTSYNQQFQDRVTITADESTSTAYMELSSLRSEDTAVYYCARDGYDDGPYTMDYWGQGTLVTVSSASTKGPSVFPLAPSSKSTSGGTAALGCLVKDYFPEPVTVSWNSGALTSGVHTFPAVLQSSGLYSLSSVVTVPSSNFGTQTYTCNVDHKPSNTKVDKTVERKSCVECPPCPAPPVAGPSVFLFPPKPKDTLMISRTPEVTCVVVDVSQEDPEVQFNWYVDGVEVHNAKTKPREEQFNSTFRVVSVLTVVHQDWLNGKEYKCKVSNKGLPAPIEKTISKTKGQPREPQVYTLPPSQEEMTKNQVSLTCLVKGFYPSDIAVEWESNGQPENNYKTTPPMLDSDGSFFLYSKLTVDKSRWQEGNVFSCSVMHEALHNHYTQKSLSLSP

SEQ ID NO: 246 - protein, 514 aa, Homo sapiens
MMWTWALWMLPSLCKFSLAALPAKPENISCVYYYRKNLTCTWSPGKETSYTQYTVKRTYAFGEKHDNCTTNSSTSENRASCSFFLPRITIPDNYTIEVEAENGDGVIKSHMTYWRLENIAKTEPPKIFRVKPVLGIKRMIQIEWIKPELAPVSSDLKYTLRFRTVNSTSWMEVNFAKNRKDKNQTYNLTGLQPFTEYVIALRCAVKESKFWSDWSQEKMGMTEEEAPCGLELWRVLKPAEADGRRPVRLLWKKARGAPVLEKTLGYNIWYYPESNTNLTETMNTTNQQLELHLGGESFWVSMISYNSLGKSPVATLRIPAIQEKSFQCIEVMQACVAEDQLVVKWQSSALDVNTWMIEWFPDVDSEPTTLSWESVSQATNWTIQQDKLKPFWCYNISVYPMLHDKVGEPYSIQAYAKEGVPSEGPETKVENIGVKTVTITWKEIPKSERKGIICNYTIFYQAEGGKGFSKTVNSSILQYGLESLKRKTSYIVQVMASTSAGGTNGTSINFKTLS